European Patent Specification EP 3 717 646 B1, published April 23, 2025. Title: ANGELMAN SYNDROME ANTISENSE TREATMENT. Applicant: The Texas A&M University System. The sequence listing filed with the application follows.

SEQUENCE LISTING (603 sequences)

SEQ ID NO: 1 - DNA, 184 bp, Artificial Sequence
  Synthetic Construct
atgatgatatggaagaaaagcactctttggcctgttgtgactgggacagttgacagcacccaggtgtcctttaatgaaaatgctcttgacaccaatgcatcctagcatcacagcttcaggaagccttctcaagtgtgcatggggagtactatgtctttcatcaataatgaaatcttctgatttg

SEQ ID NO: 2 - DNA, 133 bp, Artificial Sequence
  Synthetic Construct
taagacatgctgccaagagatgtgccattctattataaaagatcagtagcttcctttaccgacgtgtatattctatctagaacattgagctatggaagactcccacctaagggaattagttttacaccttcag

SEQ ID NO: 3 - DNA, 125 bp, Artificial Sequence
  Synthetic Construct
ataaagactgctgagaagagcaccctctggtgttgtcacagaggcaagtgctaccgcacaggcatgctgcagtgaatttaactgatcctctgtccctgcaaccgttgtttaaggatgctattctg

SEQ ID NO: 4 - DNA, 129 bp, Artificial Sequence
  Synthetic Construct
aaaagactgtggaggaagaaaaccctttaccctgttgttcagggagaaactgacaccactcaactgcctggcactgaaaatgtggcatccagtccactttaccatcagtgtttaaggaaaccatctctg

SEQ ID NO: 5 - DNA, 117 bp, Artificial Sequence
  Synthetic Construct
ataaggatgactgaggaagagtactctttggcttgttgacaccagcacagctgacacacccagatatctgtttggtctcctgtgaactttcaaccaggatttaaggatgccactctg

SEQ ID NO: 6 - DNA, 20 bp, Artificial Sequence
  Synthetic Construct
tagaggtgaaggccaggcac

SEQ ID NO: 7 - DNA, 20 bp, Artificial Sequence
  Synthetic Construct
gtactcttcctcagtcatcc

SEQ ID NO: 8 - DNA, 20 bp, Artificial Sequence
  Synthetic Construct
tgtcagtttctccctgaaca

SEQ ID NO: 9 - DNA, 20 bp, Artificial Sequence
  Synthetic Construct
tagaatggcacatctcttgg

SEQ ID NO: 10 - DNA, 20 bp, Artificial Sequence
  Synthetic Construct
gttttcttcctccacagtct

SEQ ID NO: 11 - DNA, 20 bp, Artificial Sequence
  Synthetic Construct
ctggtgtcaacaagccaaag

SEQ ID NO: 12 - RNA, 18 nt, Artificial Sequence
  Synthetic Construct
gaaaaugcucuugacacc

SEQ ID NO: 13 - RNA, 19 nt, Artificial Sequence
  Synthetic Construct
gaaaaugcucuugacacca

SEQ ID NO: 14 - RNA, 20 nt, Artificial Sequence
  Synthetic Construct
gaaaaugcucuugacaccaa

SEQ ID NO: 15 - DNA, 18 bp, Artificial Sequence
  Synthetic Construct
ggtgtcaagagcattttc

SEQ ID NO: 16 - DNA, 19 bp, Artificial Sequence
  Synthetic Construct
tggtgtcaagagcattttc

SEQ ID NO: 17 - DNA, 20 bp, Artificial Sequence
  Synthetic Construct
ttggtgtcaagagcattttc

SEQ ID NO: 18 - RNA, 18 nt, Artificial Sequence
  Synthetic Construct
caugcugccaagagaugu

SEQ ID NO: 19 - RNA, 19 nt, Artificial Sequence
  Synthetic Construct
caugcugccaagagaugug

SEQ ID NO: 20 - RNA, 20 nt, Artificial Sequence
  Synthetic Construct
caugcugccaagagaugugc

SEQ ID NO: 21 - RNA, 18 nt, Artificial Sequence
  Synthetic Construct
augcugccaagagaugug

SEQ ID NO: 22 - RNA, 19 nt, Artificial Sequence
  Synthetic Construct
augcugccaagagaugugc

SEQ ID NO: 23 - RNA, 20 nt, Artificial Sequence
  Synthetic Construct
augcugccaagagaugugcc

SEQ ID NO: 24 - RNA, 19 nt, Artificial Sequence
  Synthetic Construct
ugcugccaagagaugugcc

SEQ ID NO: 25 - RNA, 20 nt, Artificial Sequence
  Synthetic Construct
ugcugccaagagaugugcca

SEQ ID NO: 26 - RNA, 19 nt, Artificial Sequence
  Synthetic Construct
gcugccaagagaugugcca

SEQ ID NO: 27 - RNA, 20 nt, Artificial Sequence
  Synthetic Construct
gcugccaagagaugugccau

SEQ ID NO: 28 - RNA, 18 nt, Artificial Sequence
  Synthetic Construct
cugccaagagaugugcca

SEQ ID NO: 29 - RNA, 19 nt, Artificial Sequence
  Synthetic Construct
cugccaagagaugugccau

SEQ ID NO: 30 - RNA, 20 nt, Artificial Sequence
  Synthetic Construct
cugccaagagaugugccauu

SEQ ID NO: 31 - RNA, 18 nt, Artificial Sequence
  Synthetic Construct
ugccaagagaugugccau

SEQ ID NO: 32 - RNA, 19 nt, Artificial Sequence
  Synthetic Construct
ugccaagagaugugccauu

SEQ ID NO: 33 - RNA, 20 nt, Artificial Sequence
  Synthetic Construct
ugccaagagaugugccauuc

SEQ ID NO: 34 - RNA, 18 nt, Artificial Sequence
  Synthetic Construct
gccaagagaugugccauu

SEQ ID NO: 35 - RNA, 19 nt, Artificial Sequence
  Synthetic Construct
gccaagagaugugccauuc

SEQ ID NO: 36 - RNA, 20 nt, Artificial Sequence
  Synthetic Construct
gccaagagaugugccauucu

SEQ ID NO: 37 - RNA, 18 nt, Artificial Sequence
  Synthetic Construct
ccaagagaugugccauuc

SEQ ID NO: 38 - RNA, 19 nt, Artificial Sequence
  Synthetic Construct
ccaagagaugugccauucu

SEQ ID NO: 39 - RNA, 20 nt, Artificial Sequence
  Synthetic Construct
ccaagagaugugccauucua

SEQ ID NO: 40 - RNA, 18 nt, Artificial Sequence
  Synthetic Construct
caagagaugugccauucu

SEQ ID NO: 41 - RNA, 19 nt, Artificial Sequence
  Synthetic Construct
caagagaugugccauucua

SEQ ID NO: 42 - RNA, 20 nt, Artificial Sequence
  Synthetic Construct
caagagaugugccauucuau

SEQ ID NO: 43 - RNA, 18 nt, Artificial Sequence
  Synthetic Construct
uccuuuaccgacguguau

SEQ ID NO: 44 - RNA, 19 nt, Artificial Sequence
  Synthetic Construct
uccuuuaccgacguguaua

SEQ ID NO: 45 - RNA, 20 nt, Artificial Sequence
  Synthetic Construct
uccuuuaccgacguguauau

SEQ ID NO: 46 - RNA, 18 nt, Artificial Sequence
  Synthetic Construct
ccuuuaccgacguguaua

SEQ ID NO: 47 - RNA, 19 nt, Artificial Sequence
  Synthetic Construct
ccuuuaccgacguguauau

SEQ ID NO: 48 - RNA, 20 nt, Artificial Sequence
  Synthetic Construct
ccuuuaccgacguguauauu

SEQ ID NO: 49 - RNA, 20 nt, Artificial Sequence
  Synthetic Construct
accgacguguauauucuauc

SEQ ID NO: 50 - RNA, 19 nt, Artificial Sequence
  Synthetic Construct
ccgacguguauauucuauc

SEQ ID NO: 51 - RNA, 20 nt, Artificial Sequence
  Synthetic Construct
ccgacguguauauucuaucu

SEQ ID NO: 52 - RNA, 20 nt, Artificial Sequence
  Synthetic Construct
ucuagaacauugagcuaugg

SEQ ID NO: 53 - RNA, 18 nt, Artificial Sequence
  Synthetic Construct
cauugagcuauggaagac

SEQ ID NO: 54 - RNA, 20 nt, Artificial Sequence
  Synthetic Construct
cuauggaagacucccaccua

SEQ ID NO: 55 - RNA, 19 nt, Artificial Sequence
  Synthetic Construct
uauggaagacucccaccua

SEQ ID NO: 56 - RNA, 20 nt, Artificial Sequence
  Synthetic Construct
uauggaagacucccaccuaa

SEQ ID NO: 57 - RNA, 18 nt, Artificial Sequence
  Synthetic Construct
auggaagacucccaccua

SEQ ID NO: 58 - RNA, 19 nt, Artificial Sequence
  Synthetic Construct
auggaagacucccaccuaa

SEQ ID NO: 59 - RNA, 18 nt, Artificial Sequence
  Synthetic Construct
uggaagacucccaccuaa

SEQ ID NO: 60 - RNA, 20 nt, Artificial Sequence
  Synthetic Construct
gacucccaccuaagggaauu

SEQ ID NO: 61 - RNA, 18 nt, Artificial Sequence
  Synthetic Construct
acucccaccuaagggaau

SEQ ID NO: 62 - RNA, 19 nt, Artificial Sequence
  Synthetic Construct
acucccaccuaagggaauu

SEQ ID NO: 63 - RNA, 20 nt, Artificial Sequence
  Synthetic Construct
acucccaccuaagggaauua

SEQ ID NO: 64 - RNA, 18 nt, Artificial Sequence
  Synthetic Construct
cucccaccuaagggaauu

SEQ ID NO: 65 - RNA, 19 nt, Artificial Sequence
  Synthetic Construct
cucccaccuaagggaauua

SEQ ID NO: 66 - RNA, 18 nt, Artificial Sequence
  Synthetic Construct
ucccaccuaagggaauua

SEQ ID NO: 67 - DNA, 18 bp, Artificial Sequence
  Synthetic Construct
acatctcttggcagcatg

SEQ ID NO: 68 - DNA, 19 bp, Artificial Sequence
  Synthetic Construct
cacatctcttggcagcatg

SEQ ID NO: 69 - DNA, 20 bp, Artificial Sequence
  Synthetic Construct
gcacatctcttggcagcatg

SEQ ID NO: 70 - DNA, 18 bp, Artificial Sequence
  Synthetic Construct
cacatctcttggcagcat

SEQ ID NO: 71 - DNA, 19 bp, Artificial Sequence
  Synthetic Construct
gcacatctcttggcagcat

SEQ ID NO: 72 - DNA, 20 bp, Artificial Sequence
  Synthetic Construct
ggcacatctcttggcagcat

SEQ ID NO: 73 - DNA, 19 bp, Artificial Sequence
  Synthetic Construct
ggcacatctcttggcagca

SEQ ID NO: 74 - DNA, 20 bp, Artificial Sequence
  Synthetic Construct
tggcacatctcttggcagca

SEQ ID NO: 75 - DNA, 19 bp, Artificial Sequence
  Synthetic Construct
tggcacatctcttggcagc

SEQ ID NO: 76 - DNA, 20 bp, Artificial Sequence
  Synthetic Construct
atggcacatctcttggcagc

SEQ ID NO: 77 - DNA, 18 bp, Artificial Sequence
  Synthetic Construct
tggcacatctcttggcag

SEQ ID NO: 78 - DNA, 19 bp, Artificial Sequence
  Synthetic Construct
atggcacatctcttggcag

SEQ ID NO: 79 - DNA, 20 bp, Artificial Sequence
  Synthetic Construct
aatggcacatctcttggcag

SEQ ID NO: 80 - DNA, 18 bp, Artificial Sequence
  Synthetic Construct
atggcacatctcttggca

SEQ ID NO: 81 - DNA, 19 bp, Artificial Sequence
  Synthetic Construct
aatggcacatctcttggca

SEQ ID NO: 82 - DNA, 20 bp, Artificial Sequence
  Synthetic Construct
gaatggcacatctcttggca

SEQ ID NO: 83 - DNA, 18 bp, Artificial Sequence
  Synthetic Construct
aatggcacatctcttggc

SEQ ID NO: 84 - DNA, 19 bp, Artificial Sequence
  Synthetic Construct
gaatggcacatctcttggc

SEQ ID NO: 85 - DNA, 20 bp, Artificial Sequence
  Synthetic Construct
agaatggcacatctcttggc

SEQ ID NO: 86 - DNA, 18 bp, Artificial Sequence
  Synthetic Construct
gaatggcacatctcttgg

SEQ ID NO: 87 - DNA, 19 bp, Artificial Sequence
  Synthetic Construct
agaatggcacatctcttgg

SEQ ID NO: 88 - DNA, 20 bp, Artificial Sequence
  Synthetic Construct
tagaatggcacatctcttgg

SEQ ID NO: 89 - DNA, 18 bp, Artificial Sequence
  Synthetic Construct
agaatggcacatctcttg

SEQ ID NO: 90 - DNA, 19 bp, Artificial Sequence
  Synthetic Construct
tagaatggcacatctcttg

SEQ ID NO: 91 - DNA, 20 bp, Artificial Sequence
  Synthetic Construct
atagaatggcacatctcttg

SEQ ID NO: 92 - DNA, 18 bp, Artificial Sequence
  Synthetic Construct
atacacgtcggtaaagga

SEQ ID NO: 93 - DNA, 19 bp, Artificial Sequence
  Synthetic Construct
tatacacgtcggtaaagga

SEQ ID NO: 94 - DNA, 20 bp, Artificial Sequence
  Synthetic Construct
atatacacgtcggtaaagga

SEQ ID NO: 95 - DNA, 18 bp, Artificial Sequence
  Synthetic Construct
tatacacgtcggtaaagg

SEQ ID NO: 96 - DNA, 19 bp, Artificial Sequence
  Synthetic Construct
atatacacgtcggtaaagg

SEQ ID NO: 97 - DNA, 20 bp, Artificial Sequence
  Synthetic Construct
aatatacacgtcggtaaagg

SEQ ID NO: 98 - DNA, 20 bp, Artificial Sequence
  Synthetic Construct
gatagaatatacacgtcggt

SEQ ID NO: 99 - DNA, 19 bp, Artificial Sequence
  Synthetic Construct
gatagaatatacacgtcgg

SEQ ID NO: 100 - DNA, 20 bp, Artificial Sequence
  Synthetic Construct
agatagaatatacacgtcgg

SEQ ID NO: 101 - DNA, 20 bp, Artificial Sequence
  Synthetic Construct
ccatagctcaatgttctaga

SEQ ID NO: 102 - DNA, 18 bp, Artificial Sequence
  Synthetic Construct
gtcttccatagctcaatg

SEQ ID NO: 103 - DNA, 20 bp, Artificial Sequence
  Synthetic Construct
taggtgggagtcttccatag

SEQ ID NO: 104 - DNA, 19 bp, Artificial Sequence
  Synthetic Construct
taggtgggagtcttccata

SEQ ID NO: 105 - DNA, 20 bp, Artificial Sequence
  Synthetic Construct
ttaggtgggagtcttccata

SEQ ID NO: 106 - DNA, 18 bp, Artificial Sequence
  Synthetic Construct
taggtgggagtcttccat

SEQ ID NO: 107 - DNA, 19 bp, Artificial Sequence
  Synthetic Construct
ttaggtgggagtcttccat

SEQ ID NO: 108 - DNA, 18 bp, Artificial Sequence
  Synthetic Construct
ttaggtgggagtcttcca

SEQ ID NO: 109 - DNA, 20 bp, Artificial Sequence
  Synthetic Construct
aattcccttaggtgggagtc

SEQ ID NO: 110 - DNA, 18 bp, Artificial Sequence
  Synthetic Construct
attcccttaggtgggagt

SEQ ID NO: 111 - DNA, 19 bp, Artificial Sequence
  Synthetic Construct
aattcccttaggtgggagt

SEQ ID NO: 112 - DNA, 20 bp, Artificial Sequence
  Synthetic Construct
taattcccttaggtgggagt

SEQ ID NO: 113 - DNA, 18 bp, Artificial Sequence
  Synthetic Construct
aattcccttaggtgggag

SEQ ID NO: 114 - DNA, 19 bp, Artificial Sequence
  Synthetic Construct
taattcccttaggtgggag

SEQ ID NO: 115 - DNA, 18 bp, Artificial Sequence
  Synthetic Construct
taattcccttaggtggga

SEQ ID NO: 116 - RNA, 20 nt, Artificial Sequence
  Synthetic Construct
gauaaagacugcugagaaga

SEQ ID NO: 117 - RNA, 20 nt, Artificial Sequence
  Synthetic Construct
auaaagacugcugagaagag

SEQ ID NO: 118 - RNA, 20 nt, Artificial Sequence
  Synthetic Construct
uaaagacugcugagaagagc

SEQ ID NO: 119 - RNA, 20 nt, Artificial Sequence
  Synthetic Construct
aaagacugcugagaagagca

SEQ ID NO: 120 - RNA, 20 nt, Artificial Sequence
  Synthetic Construct
aagacugcugagaagagcac

SEQ ID NO: 121 - RNA, 20 nt, Artificial Sequence
  Synthetic Construct
agacugcugagaagagcacc

SEQ ID NO: 122 - RNA, 20 nt, Artificial Sequence
  Synthetic Construct
gacugcugagaagagcaccc

SEQ ID NO: 123 - RNA, 20 nt, Artificial Sequence
  Synthetic Construct
caagugcuaccgcacaggca

SEQ ID NO: 124 - RNA, 20 nt, Artificial Sequence
  Synthetic Construct
aagugcuaccgcacaggcau

SEQ ID NO: 125 - RNA, 20 nt, Artificial Sequence
  Synthetic Construct
agugcuaccgcacaggcaug

SEQ ID NO: 126 - RNA, 20 nt, Artificial Sequence
  Synthetic Construct
ugcuaccgcacaggcaugcu

SEQ ID NO: 127 - RNA, 20 nt, Artificial Sequence
  Synthetic Construct
uaccgcacaggcaugcugca

SEQ ID NO: 128 - RNA, 20 nt, Artificial Sequence
  Synthetic Construct
gcacaggcaugcugcaguga

SEQ ID NO: 129 - RNA, 20 nt, Artificial Sequence
  Synthetic Construct
cacaggcaugcugcagugaa

SEQ ID NO: 130 - RNA, 20 nt, Artificial Sequence
  Synthetic Construct
acaggcaugcugcagugaau

SEQ ID NO: 131 - RNA, 20 nt, Artificial Sequence
  Synthetic Construct
caggcaugcugcagugaauu

SEQ ID NO: 132 - RNA, 20 nt, Artificial Sequence
  Synthetic Construct
aggcaugcugcagugaauuu

SEQ ID NO: 133 - RNA, 20 nt, Artificial Sequence
  Synthetic Construct
ggcaugcugcagugaauuua

SEQ ID NO: 134 - RNA, 20 nt, Artificial Sequence
  Synthetic Construct
gcaugcugcagugaauuuaa

SEQ ID NO: 135 - RNA, 20 nt, Artificial Sequence
  Synthetic Construct
caugcugcagugaauuuaac

SEQ ID NO: 136 - RNA, 20 nt, Artificial Sequence
  Synthetic Construct
gcagugaauuuaacugaucc

SEQ ID NO: 137 - RNA, 20 nt, Artificial Sequence
  Synthetic Construct
ucccugcaaccguuguuuaa

SEQ ID NO: 138 - RNA, 20 nt, Artificial Sequence
  Synthetic Construct
cccugcaaccguuguuuaag

SEQ ID NO: 139 - DNA, 20 bp, Artificial Sequence
  Synthetic Construct
tcttctcagcagtctttatc

SEQ ID NO: 140 - DNA, 20 bp, Artificial Sequence
  Synthetic Construct
ctcttctcagcagtctttat

SEQ ID NO: 141 - DNA, 20 bp, Artificial Sequence
  Synthetic Construct
gctcttctcagcagtcttta

SEQ ID NO: 142 - DNA, 20 bp, Artificial Sequence
  Synthetic Construct
tgctcttctcagcagtcttt

SEQ ID NO: 143 - DNA, 20 bp, Artificial Sequence
  Synthetic Construct
gtgctcttctcagcagtctt

SEQ ID NO: 144 - DNA, 20 bp, Artificial Sequence
  Synthetic Construct
ggtgctcttctcagcagtct

SEQ ID NO: 145 - DNA, 20 bp, Artificial Sequence
  Synthetic Construct
gggtgctcttctcagcagtc

SEQ ID NO: 146 - DNA, 20 bp, Artificial Sequence
  Synthetic Construct
tgcctgtgcggtagcacttg

SEQ ID NO: 147 - DNA, 20 bp, Artificial Sequence
  Synthetic Construct
atgcctgtgcggtagcactt

SEQ ID NO: 148 - DNA, 20 bp, Artificial Sequence
  Synthetic Construct
catgcctgtgcggtagcact

SEQ ID NO: 149 - DNA, 20 bp, Artificial Sequence
  Synthetic Construct
agcatgcctgtgcggtagca

SEQ ID NO: 150 - DNA, 20 bp, Artificial Sequence
  Synthetic Construct
tgcagcatgcctgtgcggta

SEQ ID NO: 151 - DNA, 20 bp, Artificial Sequence
  Synthetic Construct
tcactgcagcatgcctgtgc

SEQ ID NO: 152 - DNA, 20 bp, Artificial Sequence
  Synthetic Construct
ttcactgcagcatgcctgtg

SEQ ID NO: 153 - DNA, 20 bp, Artificial Sequence
  Synthetic Construct
attcactgcagcatgcctgt

SEQ ID NO: 154 - DNA, 20 bp, Artificial Sequence
  Synthetic Construct
aattcactgcagcatgcctg

SEQ ID NO: 155 - DNA, 20 bp, Artificial Sequence
  Synthetic Construct
aaattcactgcagcatgcct

SEQ ID NO: 156 - DNA, 20 bp, Artificial Sequence
  Synthetic Construct
taaattcactgcagcatgcc

SEQ ID NO: 157 - DNA, 20 bp, Artificial Sequence
  Synthetic Construct
ttaaattcactgcagcatgc

SEQ ID NO: 158 - DNA, 20 bp, Artificial Sequence
  Synthetic Construct
gttaaattcactgcagcatg

SEQ ID NO: 159 - DNA, 20 bp, Artificial Sequence
  Synthetic Construct
ggatcagttaaattcactgc

SEQ ID NO: 160 - DNA, 20 bp, Artificial Sequence
  Synthetic Construct
ttaaacaacggttgcaggga

SEQ ID NO: 161 - DNA, 20 bp, Artificial Sequence
  Synthetic Construct
cttaaacaacggttgcaggg

SEQ ID NO: 162 - RNA, 19 nt, Artificial Sequence
  Synthetic Construct
aaaagacuguggaggaaga

SEQ ID NO: 163 - RNA, 20 nt, Artificial Sequence
  Synthetic Construct
aaaagacuguggaggaagaa

SEQ ID NO: 164 - RNA, 19 nt, Artificial Sequence
  Synthetic Construct
aaagacuguggaggaagaa

SEQ ID NO: 165 - RNA, 20 nt, Artificial Sequence
  Synthetic Construct
aaagacuguggaggaagaaa

SEQ ID NO: 166 - RNA, 20 nt, Artificial Sequence
  Synthetic Construct
aagacuguggaggaagaaaa

SEQ ID NO: 167 - RNA, 20 nt, Artificial Sequence
  Synthetic Construct
agacuguggaggaagaaaac

SEQ ID NO: 168 - RNA, 18 nt, Artificial Sequence
  Synthetic Construct
acuguggaggaagaaaac

SEQ ID NO: 169 - RNA, 19 nt, Artificial Sequence
  Synthetic Construct
acuguggaggaagaaaacc

SEQ ID NO: 170 - RNA, 20 nt, Artificial Sequence
  Synthetic Construct
acuguggaggaagaaaaccc

SEQ ID NO: 171 - RNA, 18 nt, Artificial Sequence
  Synthetic Construct
cuguggaggaagaaaacc

SEQ ID NO: 172 - RNA, 19 nt, Artificial Sequence
  Synthetic Construct
cuguggaggaagaaaaccc

SEQ ID NO: 173 - RNA, 19 nt, Artificial Sequence
  Synthetic Construct
aaaacccuuuacccuguug

SEQ ID NO: 174 - RNA, 20 nt, Artificial Sequence
  Synthetic Construct
aaaacccuuuacccuguugu

SEQ ID NO: 175 - RNA, 20 nt, Artificial Sequence
  Synthetic Construct
aaacccuuuacccuguuguu

SEQ ID NO: 176 - RNA, 18 nt, Artificial Sequence
  Synthetic Construct
uuguucagggagaaacug

SEQ ID NO: 177 - RNA, 20 nt, Artificial Sequence
  Synthetic Construct
uuguucagggagaaacugac

SEQ ID NO: 178 - RNA, 18 nt, Artificial Sequence
  Synthetic Construct
uguucagggagaaacuga

SEQ ID NO: 179 - RNA, 19 nt, Artificial Sequence
  Synthetic Construct
uguucagggagaaacugac

SEQ ID NO: 180 - RNA, 20 nt, Artificial Sequence
  Synthetic Construct
uguucagggagaaacugaca

SEQ ID NO: 181 - RNA, 19 nt, Artificial Sequence
  Synthetic Construct
guucagggagaaacugaca

SEQ ID NO: 182 - RNA, 20 nt, Artificial Sequence
  Synthetic Construct
ucagggagaaacugacacca

SEQ ID NO: 183 - RNA, 19 nt, Artificial Sequence
  Synthetic Construct
cagggagaaacugacacca

SEQ ID NO: 184 - RNA, 18 nt, Artificial Sequence
  Synthetic Construct
agggagaaacugacacca

SEQ ID NO: 185 - RNA, 19 nt, Artificial Sequence
  Synthetic Construct
agggagaaacugacaccac

SEQ ID NO: 186 - RNA, 20 nt, Artificial Sequence
  Synthetic Construct
agggagaaacugacaccacu

SEQ ID NO: 187 - RNA, 18 nt, Artificial Sequence
  Synthetic Construct
gggagaaacugacaccac

SEQ ID NO: 188 - RNA, 19 nt, Artificial Sequence
  Synthetic Construct
gggagaaacugacaccacu

SEQ ID NO: 189 - RNA, 20 nt, Artificial Sequence
  Synthetic Construct
gggagaaacugacaccacuc

SEQ ID NO: 190 - RNA, 18 nt, Artificial Sequence
  Synthetic Construct
ggagaaacugacaccacu

SEQ ID NO: 191 - RNA, 19 nt, Artificial Sequence
  Synthetic Construct
ggagaaacugacaccacuc

SEQ ID NO: 192 - RNA, 20 nt, Artificial Sequence
  Synthetic Construct
ggagaaacugacaccacuca

SEQ ID NO: 193 - RNA, 18 nt, Artificial Sequence
  Synthetic Construct
gagaaacugacaccacuc

SEQ ID NO: 194 - RNA, 19 nt, Artificial Sequence
  Synthetic Construct
gagaaacugacaccacuca

SEQ ID NO: 195 - RNA, 20 nt, Artificial Sequence
  Synthetic Construct
gagaaacugacaccacucaa

SEQ ID NO: 196 - RNA, 18 nt, Artificial Sequence
  Synthetic Construct
agaaacugacaccacuca

SEQ ID NO: 197 - RNA, 19 nt, Artificial Sequence
  Synthetic Construct
agaaacugacaccacucaa

SEQ ID NO: 198 - RNA, 20 nt, Artificial Sequence
  Synthetic Construct
agaaacugacaccacucaac

SEQ ID NO: 199 - RNA, 18 nt, Artificial Sequence
  Synthetic Construct
gaaacugacaccacucaa

SEQ ID NO: 200 - RNA, 19 nt, Artificial Sequence
  Synthetic Construct
gaaacugacaccacucaac

SEQ ID NO: 201 - RNA, 20 nt, Artificial Sequence
  Synthetic Construct
gaaacugacaccacucaacu

SEQ ID NO: 202 - RNA, 18 nt, Artificial Sequence
  Synthetic Construct
aaacugacaccacucaac

SEQ ID NO: 203 - RNA, 19 nt, Artificial Sequence
  Synthetic Construct
aaacugacaccacucaacu

SEQ ID NO: 204 - RNA, 20 nt, Artificial Sequence
  Synthetic Construct
aaacugacaccacucaacug

SEQ ID NO: 205 - RNA, 18 nt, Artificial Sequence
  Synthetic Construct
aacugacaccacucaacu

SEQ ID NO: 206 - RNA, 19 nt, Artificial Sequence
  Synthetic Construct
aacugacaccacucaacug

SEQ ID NO: 207 - RNA, 20 nt, Artificial Sequence
  Synthetic Construct
aacugacaccacucaacugc

SEQ ID NO: 208 - RNA, 18 nt, Artificial Sequence
  Synthetic Construct
acugacaccacucaacug

SEQ ID NO: 209 - RNA, 19 nt, Artificial Sequence
  Synthetic Construct
acugacaccacucaacugc

SEQ ID NO: 210 - RNA, 20 nt, Artificial Sequence
  Synthetic Construct
acugacaccacucaacugcc

SEQ ID NO: 211 - RNA, 18 nt, Artificial Sequence
  Synthetic Construct
cugacaccacucaacugc

SEQ ID NO: 212 - RNA, 19 nt, Artificial Sequence
  Synthetic Construct
cugacaccacucaacugcc

SEQ ID NO: 213 - RNA, 20 nt, Artificial Sequence
  Synthetic Construct
cugacaccacucaacugccu

SEQ ID NO: 214 - RNA, 18 nt, Artificial Sequence
  Synthetic Construct
ugacaccacucaacugcc

SEQ ID NO: 215 - RNA, 19 nt, Artificial Sequence
  Synthetic Construct
ugacaccacucaacugccu

SEQ ID NO: 216 - RNA, 20 nt, Artificial Sequence
  Synthetic Construct
ugacaccacucaacugccug

SEQ ID NO: 217 - RNA, 18 nt, Artificial Sequence
  Synthetic Construct
gacaccacucaacugccu

SEQ ID NO: 218 - RNA, 19 nt, Artificial Sequence
  Synthetic Construct
gacaccacucaacugccug

SEQ ID NO: 219 - RNA, 20 nt, Artificial Sequence
  Synthetic Construct
gacaccacucaacugccugg

SEQ ID NO: 220 - RNA, 18 nt, Artificial Sequence
  Synthetic Construct
acaccacucaacugccug

SEQ ID NO: 221 - RNA, 19 nt, Artificial Sequence
  Synthetic Construct
acaccacucaacugccugg

SEQ ID NO: 222 - RNA, 20 nt, Artificial Sequence
  Synthetic Construct
acaccacucaacugccuggc

SEQ ID NO: 223 - RNA, 20 nt, Artificial Sequence
  Synthetic Construct
caccacucaacugccuggca

SEQ ID NO: 224 - RNA, 18 nt, Artificial Sequence
  Synthetic Construct
gaaaauguggcauccagu

SEQ ID NO: 225 - RNA, 18 nt, Artificial Sequence
  Synthetic Construct
aaaauguggcauccaguc

SEQ ID NO: 226 - RNA, 20 nt, Artificial Sequence
  Synthetic Construct
gcauccaguccacuuuacca

SEQ ID NO: 227 - RNA, 18 nt, Artificial Sequence
  Synthetic Construct
cauccaguccacuuuacc

SEQ ID NO: 228 - RNA, 19 nt, Artificial Sequence
  Synthetic Construct
cauccaguccacuuuacca

SEQ ID NO: 229 - RNA, 20 nt, Artificial Sequence
  Synthetic Construct
cauccaguccacuuuaccau

SEQ ID NO: 230 - RNA, 18 nt, Artificial Sequence
  Synthetic Construct
auccaguccacuuuacca

SEQ ID NO: 231 - RNA, 19 nt, Artificial Sequence
  Synthetic Construct
auccaguccacuuuaccau

SEQ ID NO: 232 - RNA, 20 nt, Artificial Sequence
  Synthetic Construct
auccaguccacuuuaccauc

SEQ ID NO: 233 - RNA, 20 nt, Artificial Sequence
  Synthetic Construct
guuuaaggaaaccaucucug

SEQ ID NO: 234 - RNA, 20 nt, Artificial Sequence
  Synthetic Construct
uuuaaggaaaccaucucugg

SEQ ID NO: 235 - RNA, 19 nt, Artificial Sequence
  Synthetic Construct
uuaaggaaaccaucucugg

SEQ ID NO: 236 - RNA, 18 nt, Artificial Sequence
  Synthetic Construct
uaaggaaaccaucucugg

SEQ ID NO: 237 - DNA, 19 bp, Artificial Sequence
  Synthetic Construct
tcttcctccacagtctttt

SEQ ID NO: 238 - DNA, 20 bp, Artificial Sequence
  Synthetic Construct
ttcttcctccacagtctttt

SEQ ID NO: 239 - DNA, 19 bp, Artificial Sequence
  Synthetic Construct
ttcttcctccacagtcttt

SEQ ID NO: 240 - DNA, 20 bp, Artificial Sequence
  Synthetic Construct
tttcttcctccacagtcttt

SEQ ID NO: 241 - DNA, 20 bp, Artificial Sequence
  Synthetic Construct
ttttcttcctccacagtctt

SEQ ID NO: 242 - DNA, 20 bp, Artificial Sequence
  Synthetic Construct
gttttcttcctccacagtct

SEQ ID NO: 243 - DNA, 18 bp, Artificial Sequence
  Synthetic Construct
gttttcttcctccacagt

SEQ ID NO: 244 - DNA, 19 bp, Artificial Sequence
  Synthetic Construct
ggttttcttcctccacagt

SEQ ID NO: 245 - DNA, 20 bp, Artificial Sequence
  Synthetic Construct
gggttttcttcctccacagt

SEQ ID NO: 246 - DNA, 18 bp, Artificial Sequence
  Synthetic Construct
ggttttcttcctccacag

SEQ ID NO: 247 - DNA, 19 bp, Artificial Sequence
  Synthetic Construct
gggttttcttcctccacag

SEQ ID NO: 248 - DNA, 19 bp, Artificial Sequence
  Synthetic Construct
caacagggtaaagggtttt

SEQ ID NO: 249 - DNA, 20 bp, Artificial Sequence
  Synthetic Construct
acaacagggtaaagggtttt

SEQ ID NO: 250 - DNA, 20 bp, Artificial Sequence
  Synthetic Construct
aacaacagggtaaagggttt

SEQ ID NO: 251 - DNA, 18 bp, Artificial Sequence
  Synthetic Construct
cagtttctccctgaacaa

SEQ ID NO: 252 - DNA, 20 bp, Artificial Sequence
  Synthetic Construct
gtcagtttctccctgaacaa

SEQ ID NO: 253 - DNA, 18 bp, Artificial Sequence
  Synthetic Construct
tcagtttctccctgaaca

SEQ ID NO: 254 - DNA, 19 bp, Artificial Sequence
  Synthetic Construct
gtcagtttctccctgaaca

SEQ ID NO: 255 - DNA, 20 bp, Artificial Sequence
  Synthetic Construct
tgtcagtttctccctgaaca

SEQ ID NO: 256 - DNA, 19 bp, Artificial Sequence
  Synthetic Construct
tgtcagtttctccctgaac

SEQ ID NO: 257 - DNA, 20 bp, Artificial Sequence
  Synthetic Construct
tggtgtcagtttctccctga

SEQ ID NO: 258 - DNA, 19 bp, Artificial Sequence
  Synthetic Construct
tggtgtcagtttctccctg

SEQ ID NO: 259 - DNA, 18 bp, Artificial Sequence
  Synthetic Construct
tggtgtcagtttctccct

SEQ ID NO: 260 - DNA, 19 bp, Artificial Sequence
  Synthetic Construct
gtggtgtcagtttctccct

SEQ ID NO: 261 - DNA, 20 bp, Artificial Sequence
  Synthetic Construct
agtggtgtcagtttctccct

SEQ ID NO: 262 - DNA, 18 bp, Artificial Sequence
  Synthetic Construct
gtggtgtcagtttctccc

SEQ ID NO: 263 - DNA, 19 bp, Artificial Sequence
  Synthetic Construct
agtggtgtcagtttctccc

SEQ ID NO: 264 - DNA, 20 bp, Artificial Sequence
  Synthetic Construct
gagtggtgtcagtttctccc

SEQ ID NO: 265 - DNA, 18 bp, Artificial Sequence
  Synthetic Construct
agtggtgtcagtttctcc

SEQ ID NO: 266 - DNA, 19 bp, Artificial Sequence
  Synthetic Construct
gagtggtgtcagtttctcc

SEQ ID NO: 267 - DNA, 20 bp, Artificial Sequence
  Synthetic Construct
tgagtggtgtcagtttctcc

SEQ ID NO: 268 - DNA, 18 bp, Artificial Sequence
  Synthetic Construct
gagtggtgtcagtttctc

SEQ ID NO: 269 - DNA, 19 bp, Artificial Sequence
  Synthetic Construct
tgagtggtgtcagtttctc

SEQ ID NO: 270 - DNA, 20 bp, Artificial Sequence
  Synthetic Construct
ttgagtggtgtcagtttctc

SEQ ID NO: 271 - DNA, 18 bp, Artificial Sequence
  Synthetic Construct
tgagtggtgtcagtttct

SEQ ID NO: 272 - DNA, 19 bp, Artificial Sequence
  Synthetic Construct
ttgagtggtgtcagtttct

SEQ ID NO: 273 - DNA, 20 bp, Artificial Sequence
  Synthetic Construct
gttgagtggtgtcagtttct

SEQ ID NO: 274 - DNA, 18 bp, Artificial Sequence
  Synthetic Construct
ttgagtggtgtcagtttc

SEQ ID NO: 275 - DNA, 19 bp, Artificial Sequence
  Synthetic Construct
gttgagtggtgtcagtttc

SEQ ID NO: 276 - DNA, 20 bp, Artificial Sequence
  Synthetic Construct
agttgagtggtgtcagtttc

SEQ ID NO: 277 - DNA, 18 bp, Artificial Sequence
  Synthetic Construct
gttgagtggtgtcagttt

SEQ ID NO: 278 - DNA, 19 bp, Artificial Sequence
  Synthetic Construct
agttgagtggtgtcagttt

SEQ ID NO: 279 - DNA, 20 bp, Artificial Sequence
  Synthetic Construct
cagttgagtggtgtcagttt

SEQ ID NO: 280 - DNA, 18 bp, Artificial Sequence
  Synthetic Construct
agttgagtggtgtcagtt

SEQ ID NO: 281 - DNA, 19 bp, Artificial Sequence
  Synthetic Construct
cagttgagtggtgtcagtt

SEQ ID NO: 282 - DNA, 20 bp, Artificial Sequence
  Synthetic Construct
gcagttgagtggtgtcagtt

SEQ ID NO: 283 - DNA, 18 bp, Artificial Sequence
  Synthetic Construct
cagttgagtggtgtcagt

SEQ ID NO: 284 - DNA, 19 bp, Artificial Sequence
  Synthetic Construct
gcagttgagtggtgtcagt

SEQ ID NO: 285 - DNA, 20 bp, Artificial Sequence
  Synthetic Construct
ggcagttgagtggtgtcagt

SEQ ID NO: 286 - DNA, 18 bp, Artificial Sequence
  Synthetic Construct
gcagttgagtggtgtcag

SEQ ID NO: 287 - DNA, 19 bp, Artificial Sequence
  Synthetic Construct
ggcagttgagtggtgtcag

SEQ ID NO: 288 - DNA, 20 bp, Artificial Sequence
  Synthetic Construct
aggcagttgagtggtgtcag

SEQ ID NO: 289 - DNA, 18 bp, Artificial Sequence
  Synthetic Construct
ggcagttgagtggtgtca

SEQ ID NO: 290 - DNA, 19 bp, Artificial Sequence
  Synthetic Construct
aggcagttgagtggtgtca

SEQ ID NO: 291 - DNA, 20 bp, Artificial Sequence
  Synthetic Construct
caggcagttgagtggtgtca

SEQ ID NO: 292 - DNA, 18 bp, Artificial Sequence
  Synthetic Construct
aggcagttgagtggtgtc

SEQ ID NO: 293 - DNA, 19 bp, Artificial Sequence
  Synthetic Construct
caggcagttgagtggtgtc

SEQ ID NO: 294 - DNA, 20 bp, Artificial Sequence
  Synthetic Construct
ccaggcagttgagtggtgtc

SEQ ID NO: 295 - DNA, 18 bp, Artificial Sequence
  Synthetic Construct
caggcagttgagtggtgt

SEQ ID NO: 296 - DNA, 19 bp, Artificial Sequence
  Synthetic Construct
ccaggcagttgagtggtgt

SEQ ID NO: 297 - DNA, 20 bp, Artificial Sequence
  Synthetic Construct
gccaggcagttgagtggtgt

SEQ ID NO: 298 - DNA, 20 bp, Artificial Sequence
  Synthetic Construct
tgccaggcagttgagtggtg

SEQ ID NO: 299 - DNA, 18 bp, Artificial Sequence
  Synthetic Construct
actggatgccacattttc

SEQ ID NO: 300 - DNA, 18 bp, Artificial Sequence
  Synthetic Construct
gactggatgccacatttt

SEQ ID NO: 301 - DNA, 20 bp, Artificial Sequence
  Synthetic Construct
tggtaaagtggactggatgc

SEQ ID NO: 302 - DNA, 18 bp, Artificial Sequence
  Synthetic Construct
ggtaaagtggactggatg

SEQ ID NO: 303 - DNA, 19 bp, Artificial Sequence
  Synthetic Construct
tggtaaagtggactggatg

SEQ ID NO: 304 - DNA, 20 bp, Artificial Sequence
  Synthetic Construct
atggtaaagtggactggatg

SEQ ID NO: 305 - DNA, 18 bp, Artificial Sequence
  Synthetic Construct
tggtaaagtggactggat

SEQ ID NO: 306 - DNA, 19 bp, Artificial Sequence
  Synthetic Construct
atggtaaagtggactggat

SEQ ID NO: 307 - DNA, 20 bp, Artificial Sequence
  Synthetic Construct
gatggtaaagtggactggat

SEQ ID NO: 308 - DNA, 20 bp, Artificial Sequence
  Synthetic Construct
cagagatggtttccttaaac

SEQ ID NO: 309 - DNA, 20 bp, Artificial Sequence
  Synthetic Construct
ccagagatggtttccttaaa

SEQ ID NO: 310 - DNA, 19 bp, Artificial Sequence
  Synthetic Construct
ccagagatggtttccttaa

SEQ ID NO: 311 - DNA, 18 bp, Artificial Sequence
  Synthetic Construct
ccagagatggtttcctta

SEQ ID NO: 312 - RNA, 19 nt, Artificial Sequence
  Synthetic Construct
auaaggaugacugaggaag

SEQ ID NO: 313 - RNA, 20 nt, Artificial Sequence
  Synthetic Construct
auaaggaugacugaggaaga

SEQ ID NO: 314 - RNA, 18 nt, Artificial Sequence
  Synthetic Construct
uaaggaugacugaggaag

SEQ ID NO: 315 - RNA, 19 nt, Artificial Sequence
  Synthetic Construct
uaaggaugacugaggaaga

SEQ ID NO: 316 - RNA, 20 nt, Artificial Sequence
  Synthetic Construct
uaaggaugacugaggaagag

SEQ ID NO: 317 - RNA, 18 nt, Artificial Sequence
  Synthetic Construct
aaggaugacugaggaaga

SEQ ID NO: 318 - RNA, 19 nt, Artificial Sequence
  Synthetic Construct
aaggaugacugaggaagag

SEQ ID NO: 319 - RNA, 20 nt, Artificial Sequence
  Synthetic Construct
aaggaugacugaggaagagu

SEQ ID NO: 320 - RNA, 18 nt, Artificial Sequence
  Synthetic Construct
aggaugacugaggaagag

SEQ ID NO: 321 - RNA, 19 nt, Artificial Sequence
  Synthetic Construct
aggaugacugaggaagagu

SEQ ID NO: 322 - RNA, 20 nt, Artificial Sequence
  Synthetic Construct
aggaugacugaggaagagua

SEQ ID NO: 323 - RNA, 18 nt, Artificial Sequence
  Synthetic Construct
ggaugacugaggaagagu

SEQ ID NO: 324 - RNA, 19 nt, Artificial Sequence
  Synthetic Construct
ggaugacugaggaagagua

SEQ ID NO: 325 - RNA, 20 nt, Artificial Sequence
  Synthetic Construct
ggaugacugaggaagaguac

SEQ ID NO: 326 - RNA, 18 nt, Artificial Sequence
  Synthetic Construct
gaugacugaggaagagua

SEQ ID NO: 327 - RNA, 19 nt, Artificial Sequence
  Synthetic Construct
gaugacugaggaagaguac

SEQ ID NO: 328 - RNA, 20 nt, Artificial Sequence
  Synthetic Construct
gaugacugaggaagaguacu

SEQ ID NO: 329 - RNA, 18 nt, Artificial Sequence
  Synthetic Construct
augacugaggaagaguac

SEQ ID NO: 330 - RNA, 19 nt, Artificial Sequence
  Synthetic Construct
augacugaggaagaguacu

SEQ ID NO: 331 - RNA, 20 nt, Artificial Sequence
  Synthetic Construct
augacugaggaagaguacuc

SEQ ID NO: 332 - RNA, 18 nt, Artificial Sequence
  Synthetic Construct
ugacugaggaagaguacu

SEQ ID NO: 333 - RNA, 19 nt, Artificial Sequence
  Synthetic Construct
ugacugaggaagaguacuc

SEQ ID NO: 334 - RNA, 20 nt, Artificial Sequence
  Synthetic Construct
ugacugaggaagaguacucu

SEQ ID NO: 335 - DNA, 19 bp, Artificial Sequence
  Synthetic Construct
cttcctcagtcatccttat

SEQ ID NO: 336 - DNA, 20 bp, Artificial Sequence
  Synthetic Construct
tcttcctcagtcatccttat

SEQ ID NO: 337 - DNA, 18 bp, Artificial Sequence
  Synthetic Construct
cttcctcagtcatcctta

SEQ ID NO: 338 - DNA, 19 bp, Artificial Sequence
  Synthetic Construct
tcttcctcagtcatcctta

SEQ ID NO: 339 - DNA, 20 bp, Artificial Sequence
  Synthetic Construct
ctcttcctcagtcatcctta

SEQ ID NO: 340 - DNA, 18 bp, Artificial Sequence
  Synthetic Construct
tcttcctcagtcatcctt

SEQ ID NO: 341 - DNA, 19 bp, Artificial Sequence
  Synthetic Construct
ctcttcctcagtcatcctt

SEQ ID NO: 342 - DNA, 20 bp, Artificial Sequence
  Synthetic Construct
actcttcctcagtcatcctt

SEQ ID NO: 343 - DNA, 18 bp, Artificial Sequence
  Synthetic Construct
ctcttcctcagtcatcct

SEQ ID NO: 344 - DNA, 19 bp, Artificial Sequence
  Synthetic Construct
actcttcctcagtcatcct

SEQ ID NO: 345 - DNA, 20 bp, Artificial Sequence
  Synthetic Construct
tactcttcctcagtcatcct

SEQ ID NO: 346 - DNA, 18 bp, Artificial Sequence
  Synthetic Construct
actcttcctcagtcatcc

SEQ ID NO: 347 - DNA, 19 bp, Artificial Sequence
  Synthetic Construct
tactcttcctcagtcatcc

SEQ ID NO: 348 - DNA, 20 bp, Artificial Sequence
  Synthetic Construct
gtactcttcctcagtcatcc

SEQ ID NO: 349 - DNA, 18 bp, Artificial Sequence
  Synthetic Construct
tactcttcctcagtcatc

SEQ ID NO: 350 - DNA, 19 bp, Artificial Sequence
  Synthetic Construct
gtactcttcctcagtcatc

SEQ ID NO: 351 - DNA, 20 bp, Artificial Sequence
  Synthetic Construct
agtactcttcctcagtcatc

SEQ ID NO: 352 - DNA, 18 bp, Artificial Sequence
  Synthetic Construct
gtactcttcctcagtcat

SEQ ID NO: 353 - DNA, 19 bp, Artificial Sequence
  Synthetic Construct
agtactcttcctcagtcat

SEQ ID NO: 354 - DNA, 20 bp, Artificial Sequence
  Synthetic Construct
gagtactcttcctcagtcat

SEQ ID NO: 355 - DNA, 18 bp, Artificial Sequence
  Synthetic Construct
agtactcttcctcagtca

SEQ ID NO: 356 - DNA, 19 bp, Artificial Sequence
  Synthetic Construct
gagtactcttcctcagtca

SEQ ID NO: 357 - DNA, 20 bp, Artificial Sequence
  Synthetic Construct
agagtactcttcctcagtca

SEQ ID NO: 358 - DNA, 20 bp, Artificial Sequence
  Synthetic Construct
  modified_base (1)..(2): 2'-O-methylcytidine
  misc_feature (1)..(20): phosphorothioate backbone
  modified_base (3)..(3): 2'-O-methyladenosine
  modified_base (4)..(4): 2'-O-methylguanosine
  modified_base (5)..(5): 2'-O-methylcytidine
  modified_base (16)..(16): 2'-O-methyladenosine
  modified_base (17)..(17): 2'-O-methyluridine
  modified_base (18)..(18): 2'-O-methylcytidine
  modified_base (19)..(19): 2'-O-methyladenosine
  modified_base (20)..(20): 2'-O-methyluridine
nnnnncttgttggatnnnnn

SEQ ID NO: 359 - DNA, 20 bp, Artificial Sequence
  Synthetic Construct
  modified_base (1)..(2): 2'-O-methylcytidine
  misc_feature (1)..(20): phosphorothioate backbone
  modified_base (3)..(3): 2'-O-methyladenosine
  modified_base (4)..(4): 2'-O-methylcytidine
  modified_base (5)..(5): 2'-O-methyladenosine
  modified_base (16)..(16): 2'-O-methyluridine
  modified_base (17)..(18): 2'-O-methylguanosine
  modified_base (19)..(20): 2'-O-methyladenosine
nnnnntttcctctcannnnn

SEQ ID NO: 360 - DNA, 20 bp, Artificial Sequence
  Synthetic Construct
  misc_feature (1)..(20): phosphorothioate backbone
  modified_base (1)..(1): 2'-O-methylguanosine
  modified_base (2)..(2): 2'-O-methyladenosine
  modified_base (3)..(3): 2'-O-methylguanosine
  modified_base (4)..(4): 2'-O-methyluridine
  modified_base (5)..(5): 2'-O-methylguanosine
  modified_base (16)..(17): 2'-O-methyladenosine
  modified_base (18)..(18): 2'-O-methyluridine
  modified_base (19)..(19): 2'-O-methylguanosine
  modified_base (20)..(20): 2'-O-methyluridine
nnnnntttgcaaaccnnnnn

SEQ ID NO: 361 - DNA, 20 bp, Artificial Sequence
  Synthetic Construct
  modified_base (1)..(1): 2'-O-methyluridine
  misc_feature (1)..(20): phosphorothioate backbone
  modified_base (2)..(2): 2'-O-methylguanosine
  modified_base (3)..(5): 2'-O-methyluridine
  modified_base (16)..(16): 2'-O-methyluridine
  modified_base (17)..(17): 2'-O-methylcytidine
  modified_base (18)..(18): 2'-O-methyluridine
  modified_base (19)..(19): 2'-O-methylguanosine
  modified_base (20)..(20): 2'-O-methylcytidine
nnnnnctttggtgatnnnnn

SEQ ID NO: 362 - DNA, 20 bp, Artificial Sequence
  Synthetic Construct
  modified_base (1)..(1): 2'-O-methyluridine
  misc_feature (1)..(20): phosphorothioate backbone
  modified_base (2)..(2): 2'-O-methyladenosine
  modified_base (3)..(3): 2'-O-methylguanosine
  modified_base (4)..(4): 2'-O-methyladenosine
  modified_base (5)..(5): 2'-O-methylguanosine
  modified_base (16)..(17): 2'-O-methylguanosine
  modified_base (18)..(18): 2'-O-methylcytidine
  modified_base (19)..(19): 2'-O-methyladenosine
  modified_base (20)..(20): 2'-O-methylcytidine
nnnnngtgaaggccannnnn

SEQ ID NO: 363 - DNA, 20 bp, Artificial Sequence
  Synthetic Construct
  modified_base (1)..(1): 2'-O-methylguanosine
  misc_feature (1)..(20): phosphorothioate backbone
  modified_base (2)..(2): 2'-O-methyluridine
  modified_base (4)..(4): 2'-O-methylcytidine
  modified_base (5)..(5): 2'-O-methyladenosine
  modified_base (5)..(5): 2'-O-methyluridine
  modified_base (17)..(18): 2'-O-methyladenosine
  modified_base (18)..(18): 2'-O-methyluridine
  modified_base (20)..(20): 2'-O-methyladenosine
nnnnncttcctcagtnnnnn

SEQ ID NO: 364 - DNA, 20 bp, Artificial Sequence
  Synthetic Construct
  modified_base (1)..(1): 2'-O-methyluridine
  misc_feature (1)..(20): phosphorothioate backbone
  modified_base (2)..(2): 2'-O-methylguanosine
  modified_base (3)..(3): 2'-O-methyluridine
  modified_base (4)..(4): 2'-O-methylcytidine
  modified_base (5)..(5): 2'-O-methyladenosine
  modified_base (16)..(16): 2'-O-methylguanosine
  modified_base (17)..(18): 2'-O-methyladenosine
  modified_base (20)..(20): 2'-O-methyladenosine
nnnnngtttctccctnnnnn

SEQ ID NO: 365 - DNA, 20 bp, Artificial Sequence
  Synthetic Construct
  modified_base (1)..(1): 2'-O-methyluridine
  misc_feature (1)..(20): phosphorothioate backbone
  modified_base (2)..(2): 2'-O-methyladenosine
  modified_base (3)..(3): 2'-O-methylguanosine
  modified_base (4)..(5): 2'-O-methyladenosine
  modified_base (16)..(16): 2'-O-methyladenosine
  modified_base (17)..(18): 2'-O-methyluridine
  modified_base (19)..(20): 2'-O-methylguanosine
nnnnntggcacatctnnnnn

SEQ ID NO: 366 - DNA, 20 bp, Artificial Sequence
  Synthetic Construct
  modified_base (1)..(1): 2'-O-methylguanosine
  misc_feature (1)..(20): phosphorothioate backbone
  modified_base (2)..(5): 2'-O-methyluridine
  modified_base (16)..(16): 2'-O-methyladenosine
  modified_base (17)..(17): 2'-O-methylguanosine
  modified_base (18)..(18): 2'-O-methyluridine
  modified_base (19)..(19): 2'-O-methylcytidine
  modified_base (20)..(20): 2'-O-methyluridine
nnnnncttcctccacnnnnn

SEQ ID NO: 367 - DNA, 20 bp, Artificial Sequence
  Synthetic Construct
  modified_base (1)..(1): 2'-O-methylcytidine
  misc_feature (1)..(20): phosphorothioate backbone
  modified_base (2)..(2): 2'-O-methyluridine
  modified_base (3)..(4): 2'-O-methylguanosine
  modified_base (5)..(5): 2'-O-methyluridine
  modified_base (16)..(16): 2'-O-methylcytidine
  modified_base (17)..(19): 2'-O-methyladenosine
  modified_base (20)..(20): 2'-O-methylguanosine
nnnnngtcaacaagcnnnnn

SEQ ID NO: 368 - DNA, 19 bp, Artificial Sequence
  Synthetic Construct
  modified_base (1)..(1): 2'-O-methylguanosine
  misc_feature (1)..(19): phosphorothioate backbone
  modified_base (2)..(3): 2'-O-methyluridine
  modified_base (4)..(4): 2'-O-methylguanosine
  modified_base (15)..(15): 2'-O-methylguanosine
  modified_base (16)..(18): 2'-O-methyluridine
  modified_base (19)..(19): 2'-O-methylcytidine
nnnnngtggtgtcannnnn

SEQ ID NO: 369 - DNA, 18 bp, Artificial Sequence
  Synthetic Construct
  modified_base (1)..(2): 2'-O-methyluridine
  misc_feature (1)..(18): phosphorothioate backbone
  modified_base (3)..(3): 2'-O-methylguanosine
  modified_base (4)..(4): 2'-O-methyladenosine
  modified_base (15)..(17): 2'-O-methyluridine
  modified_base (18)..(18): 2'-O-methylcytidine
nnnnntggtgtcannnnn

SEQ ID NO: 370 - DNA, 18 bp, Artificial Sequence
  Synthetic Construct
  modified_base (1)..(1): 2'-O-methylcytidine
  modified_base (1)..(18): phosphorothioate backbone
  misc_feature (1)..(5): n is a, c, g, t or u
  modified_base (2)..(2): 2'-O-methyluridine
  modified_base (3)..(4): 2'-O-methylguanosine
  misc_feature (14)..(18): n is a, c, g, t or u
  modified_base (15)..(16): 2'-O-methylcytidine
  modified_base (17)..(18): 2'-O-methyladenosine
nnnnngtcaacaannnnn

SEQ ID NO: 371 - DNA, 20 bp, Artificial Sequence
  Synthetic Construct
  modified_base (1)..(1): 2'-O-methyladenosine
  misc_feature (1)..(20): phosphorothioate backbone
  modified_base (2)..(2): 2'-O-methyluridine
  modified_base (3)..(3): 2'-O-methyladenosine
  modified_base (4)..(4): 2'-O-methylguanosine
  modified_base (5)..(5): 2'-O-methyladenosine
  modified_base (16)..(16): 2'-O-methyluridine
  modified_base (17)..(17): 2'-O-methylcytidine
  modified_base (18)..(19): 2'-O-methyluridine
  modified_base (20)..(20): 2'-O-methylguanosine
nnnnnatggcacatcnnnnn

SEQ ID NO: 372 - DNA, 19 bp, Artificial Sequence
  Synthetic Construct
  modified_base (1)..(1): 2'-O-methyladenosine
  misc_feature (1)..(19): phosphorothioate backbone
  modified_base (2)..(2): 2'-O-methylguanosine
  modified_base (3)..(4): 2'-O-methyladenosine
  modified_base (15)..(15): 2'-O-methylcytidine
  modified_base (16)..(17): 2'-O-methyluridine
  modified_base (18)..(19): 2'-O-methylguanosine
nnnnnggcacatctnnnnn

SEQ ID NO: 373 - DNA, 19 bp, Artificial Sequence
  Synthetic Construct
  modified_base (1)..(1): 2'-O-methyluridine
  misc_feature (1)..(19): phosphorothioate backbone
  modified_base (2)..(2): 2'-O-methyladenosine
  modified_base (3)..(3): 2'-O-methylguanosine
  modified_base (4)..(4): 2'-O-methyladenosine
  modified_base (15)..(15): 2'-O-methyluridine
  modified_base (16)..(16): 2'-O-methylcytidine
  modified_base (17)..(18): 2'-O-methyluridine
  modified_base (19)..(19): 2'-O-methylguanosine
nnnnntggcacatcnnnnn

SEQ ID NO: 374 - DNA, 18 bp, Artificial Sequence
  Synthetic Construct
  modified_base (1)..(1): 2'-O-methyladenosine
  misc_feature (1)..(18): phosphorothioate backbone
  modified_base (2)..(2): 2'-O-methylguanosine
  modified_base (3)..(4): 2'-O-methyladenosine
  modified_base (15)..(15): 2'-O-methylcytidine
  modified_base (16)..(17): 2'-O-methyluridine
  modified_base (18)..(18): 2'-O-methylguanosine
nnnnnggcacatcnnnnn

SEQ ID NO: 375 - DNA, 20 bp, Artificial Sequence
  Synthetic Construct
  modified_base (1)..(1): 2'-O-methyluridine
  misc_feature (1)..(20): phosphorothioate backbone
  modified_base (2)..(2): 2'-O-methyladenosine
  modified_base (3)..(3): 2'-O-methylguanosine
  modified_base (4)..(5): 2'-O-methyladenosine
  modified_base (16)..(16): 2'-O-methylcytidine
  modified_base (17)..(18): 2'-O-methyluridine
  modified_base (19)..(20): 2'-O-methylguanosine
nnnnntggcacatctnnnnn

SEQ ID NO: 376 - DNA, 20 bp, Artificial Sequence
  Synthetic Construct
  modified_base (1)..(1): 2'-O-methyluridine
  misc_feature (1)..(5): phosphorothioate backbone
  modified_base (2)..(2): 2'-O-methyladenosine
  modified_base (3)..(3): 2'-O-methylguanosine
  modified_base (4)..(5): 2'-O-methyladenosine
  misc_feature (5)..(6): phosphodiester backbone
  misc_feature (6)..(15): phosphorothioate backbone
  misc_feature (15)..(16): phosphodiester backbone
  misc_feature (16)..(20): phosphorothioate backbone
  modified_base (16)..(16): 2'-O-methylcytidine
  modified_base (17)..(18): 2'-O-methyluridine
  modified_base (19)..(20): 2'-O-methylguanosine
nnnnntggcacatctnnnnn

SEQ ID NO: 377 - DNA, 20 bp, Artificial Sequence
  Synthetic Construct
  modified_base (1)..(1): 2'-O-methyluridine
  misc_feature (1)..(5): phosphorothioate backbone
  modified_base (2)..(2): 2'-O-methyladenosine
  modified_base (3)..(3): 2'-O-methylguanosine
  modified_base (4)..(5): 2'-O-methyladenosine
  misc_feature (5)..(6): phosphodiester backbone
  misc_feature (6)..(15): phosphorothioate backbone
  misc_feature (15)..(16): phosphodiester backbone
  misc_feature (16)..(20): phosphorothioate backbone
  modified_base (16)..(16): 2'-O-methylcytidine
  modified_base (17)..(18): 2'-O-methyluridine
  modified_base (19)..(20): 2'-O-methylguanosine
nnnnntggcacatctnnnnn

SEQ ID NO: 378 - DNA, 20 bp, Artificial Sequence
  Synthetic Construct
  modified_base (1)..(1): 2'-O-(2-methoxyethyl)-modified thymidine
  misc_feature (1)..(20): phosphorothioate backbone
  modified_base (2)..(2): 2'-O-(2-methoxyethyl)-modified adenosine
  modified_base (3)..(3): 2'-O-(2-methoxyethyl)-modified guanosine
  modified_base (4)..(5): 2'-O-(2-methoxyethyl)-modified adenosine
  modified_base (16)..(16): 2'-O-(2-methoxyethyl)-modified 5-methylcytidine
  modified_base (17)..(18): 2'-O-(2-methoxyethyl)-modified thymidine
  modified_base (19)..(20): 2'-O-(2-methoxyethyl)-modified guanosine
nnnnntggcacatctnnnnn

SEQ ID NO: 379 - DNA, 20 bp, Artificial Sequence
  Synthetic Construct
  misc_feature (1)..(5): phosphorothioate backbone
  modified_base (1)..(1): 2'-O-(2-methoxyethyl)-modified thymidine
  modified_base (2)..(2): 2'-O-(2-methoxyethyl)-modified adenosine
  modified_base (3)..(3): 2'-O-(2-methoxyethyl)-modified guanosine
  modified_base (4)..(5): 2'-O-(2-methoxyethyl)-modified adenosine
  misc_feature (5)..(6): phosphodiester backbone
  misc_feature (6)..(15): phosphorothioate backbone
  misc_feature (15)..(16): phosphodiester backbone
  modified_base (16)..(16): 2'-O-(2-methoxyethyl)-modified 5-methylcytidine
  misc_feature (16)..(20): phosphorothioate backbone
  modified_base (17)..(18): 2'-O-(2-methoxyethyl)-modified thymidine
  modified_base (19)..(20): 2'-O-(2-methoxyethyl)-modified guanosine
nnnnntggcacatctnnnnn

SEQ ID NO: 380 - DNA, 20 bp, Artificial Sequence
  Synthetic Construct
  modified_base (1)..(1): 2'-O-(2-methoxyethyl)-modified thymidine
  misc_feature (1)..(2): phosphorothioate backbone
  misc_feature (2)..(3): phosphodiester backbone
  modified_base (2)..(2): 2'-O-(2-methoxyethyl)-modified adenosine
  misc_feature (3)..(4): phosphorothioate backbone
  modified_base (3)..(3): 2'-O-(2-methoxyethyl)-modified guanosine
  misc_feature (4)..(5): phosphodiester backbone
  modified_base (4)..(5): 2'-O-(2-methoxyethyl)-modified adenosine
  misc_feature (5)..(6): phosphorothioate backbone
  misc_feature (6)..(7): phosphodiester backbone
  misc_feature (7)..(8): phosphorothioate backbone
  misc_feature (8)..(9): phosphodiester backbone
  misc_feature (9)..(10): phosphorothioate backbone
  misc_feature (10)..(11): phosphodiester backbone
  misc_feature (11)..(12): phosphorothioate backbone
  misc_feature (12)..(13): phosphodiester backbone
  misc_feature (13)..(14): phosphorothioate backbone
  misc_feature (14)..(15): phosphodiester backbone
  misc_feature (15)..(16): phosphorothioate backbone
  misc_feature (16)..(17): phosphodiester backbone
  modified_base (16)..(16): 2'-O-(2-methoxyethyl)-modified 5-methylcytidine
  misc_feature (17)..(18): phosphorothioate backbone
  modified_base (17)..(18): 2'-O-(2-methoxyethyl)-modified thymidine
  misc_feature (18)..(19): phosphodiester backbone
  misc_feature (19)..(20): phosphorothioate backbone
  modified_base (19)..(20): 2'-O-(2-methoxyethyl)-modified guanosine
nnnnntggcacatctnnnnn

SEQ ID NO: 381 - DNA, 18 bp, Artificial Sequence
  Synthetic Construct
  modified_base (1)..(1): locked nucleic acid adenosine
  misc_feature (1)..(18): phosphorothioate backbone
  modified_base (3)..(3): locked nucleic acid adenosine
  modified_base (15)..(15): locked nucleic acid 5-methylcytidine
  modified_base (16)..(17): locked nucleic acid thymidine
  modified_base (18)..(18): locked nucleic acid guanosine
nnnatggcacatctnnnn

SEQ ID NO: 382 - DNA, 18 bp, Artificial Sequence
  Synthetic Construct
  modified_base (1)..(1): locked nucleic acid adenosine
  misc_feature (1)..(3): phosphorothioate backbone
  modified_base (2)..(2): locked nucleic acid guanosine
  misc_feature (3)..(4): phosphodiester backbone
  modified_base (3)..(3): locked nucleic acid adenosine
  misc_feature (4)..(14): phosphorothioate backbone
  misc_feature (14)..(15): phosphodiester backbone
  misc_feature (15)..(18): phosphorothioate backbone
  modified_base (15)..(15): locked nucleic acid 5-methylcytidine
  modified_base (16)..(17): locked nucleic acid thymidine
  modified_base (18)..(18): locked nucleic acid guanosine
nnnatggcacatctnnnn

SEQ ID NO: 383 - DNA, 18 bp, Artificial Sequence
  Synthetic Construct
  modified_base (1)..(1): locked nucleic acid adenosine
  misc_feature (1)..(2): phosphorothioate backbone
  misc_feature (2)..(3): phosphodiester backbone
  modified_base (2)..(2): locked nucleic acid guanosine
  misc_feature (3)..(4): phosphorothioate backbone
  modified_base (3)..(3): locked nucleic acid adenosine
  misc_feature (4)..(5): phosphodiester backbone
  misc_feature (5)..(6): phosphorothioate backbone
  misc_feature (6)..(7): phosphodiester backbone
  misc_feature (7)..(8): phosphorothioate backbone
  misc_feature (8)..(9): phosphodiester backbone
  misc_feature (9)..(10): phosphorothioate backbone
  misc_feature (10)..(11): phosphodiester backbone
  misc_feature (11)..(12): phosphorothioate backbone
  misc_feature (12)..(13): phosphodiester backbone
  misc_feature (13)..(14): phosphorothioate backbone
  misc_feature (14)..(15): phosphodiester backbone
  misc_feature (15)..(16): phosphorothioate backbone
  modified_base (15)..(15): locked nucleic acid 5-methylcytidine
  misc_feature (16)..(17): phosphodiester backbone
  modified_base (16)..(17): locked nucleic acid thymidine
  misc_feature (17)..(18): phosphorothioate backbone
  modified_base (18)..(18): locked nucleic acid guanosine
nnnatggcacatctnnnn

SEQ ID NO: 384 - DNA, 18 bp, Artificial Sequence
  Synthetic Construct
  modified_base (1)..(1): 2'-O-methylcytidine
  misc_feature (1)..(18): phosphorothioate backbone
  modified_base (2)..(2): 2'-O-methyluridine
  modified_base (3)..(4): 2'-O-methylguanosine
  modified_base (15)..(16): 2'-O-methylcytidine
  modified_base (17)..(18): 2'-O-methyladenosine
nnnntgtcaacaagnnnn

SEQ ID NO: 385 - DNA, 18 bp, Artificial Sequence
  Synthetic Construct
  modified_base (1)..(1): 2'-O-methylcytidine
  misc_feature (1)..(4): phosphorothioate backbone
  modified_base (2)..(2): 2'-O-methyluridine
  modified_base (3)..(4): 2'-O-methylguanosine
  misc_feature (4)..(5): phosphodiester backbone
  misc_feature (5)..(14): phosphorothioate backbone
  misc_feature (14)..(15): phosphodiester backbone
  misc_feature (15)..(18): phosphorothioate backbone
  modified_base (15)..(16): 2'-O-methylcytidine
  modified_base (17)..(18): 2'-O-methyladenosine
nnnntgtcaacaagnnnn

SEQ ID NO: 386 - DNA, 18 bp, Artificial Sequence
  Synthetic Construct
  modified_base (1)..(1): 2'-O-methylcytidine
  misc_feature (1)..(2): phosphorothioate backbone
  misc_feature (2)..(3): phosphodiester backbone
  modified_base (2)..(2): 2'-O-methyluridine
  misc_feature (3)..(4): phosphorothioate backbone
  modified_base (3)..(4): 2'-O-methylguanosine
  misc_feature (4)..(5): phosphodiester backbone
  misc_feature (5)..(14): phosphorothioate backbone
  misc_feature (5)..(6): phosphorothioate backbone
  misc_feature (6)..(7): phosphodiester backbone
  misc_feature (7)..(8): phosphorothioate backbone
  misc_feature (8)..(9): phosphodiester backbone
  misc_feature (9)..(10): phosphorothioate backbone
  misc_feature (10)..(11): phosphodiester backbone
  misc_feature (11)..(12): phosphorothioate backbone
  misc_feature (12)..(13): phosphodiester backbone
  misc_feature (13)..(14): phosphorothioate backbone
  misc_feature (14)..(15): phosphodiester backbone
  misc_feature (15)..(16): phosphorothioate backbone
  modified_base (15)..(16): 2'-O-methylcytidine
  misc_feature (16)..(17): phosphodiester backbone
  misc_feature (17)..(18): phosphorothioate backbone
  modified_base (17)..(18): 2'-O-methyladenosine
nnnntgtcaacaagnnnn

SEQ ID NO: 387 - DNA, 18 bp, Artificial Sequence
  Synthetic Construct
  modified_base (1)..(1): 2'-O-(2-methoxyethyl)-modified 5-methylcytidine
  misc_feature (1)..(18): phosphorothioate backbone
  modified_base (2)..(2): 2'-O-(2-methoxyethyl)-modified thymidine
  modified_base (3)..(4): 2'-O-(2-methoxyethyl)-modified guanosine
  modified_base (15)..(16): 2'-O-(2-methoxyethyl)-modified 5-methylcytidine
  modified_base (17)..(18): 2'-O-(2-methoxyethyl)-modified adenosine
nnnntgtcaacaagnnnn

SEQ ID NO: 388 - DNA, 18 bp, Artificial Sequence
  Synthetic Construct
  modified_base (1)..(1): 2'-O-(2-methoxyethyl)-modified 5-methylcytidine
  misc_feature (1)..(4): phosphorothioate backbone
  modified_base (2)..(2): 2'-O-(2-methoxyethyl)-modified thymidine
  modified_base (3)..(4): 2'-O-(2-methoxyethyl)-modified guanosine
  misc_feature (4)..(5): phosphodiester backbone
  misc_feature (5)..(14): phosphorothioate backbone
  misc_feature (14)..(15): phosphodiester backbone
  misc_feature (15)..(18): phosphorothioate backbone
  modified_base (15)..(16): 2'-O-(2-methoxyethyl)-modified 5-methylcytidine
  modified_base (17)..(18): 2'-O-(2-methoxyethyl)-modified adenosine
nnnntgtcaacaagnnnn

SEQ ID NO: 389 - DNA, 18 bp, Artificial Sequence
  Synthetic Construct
  modified_base (1)..(1): 2'-O-(2-methoxyethyl)-modified 5-methylcytidine
  misc_feature (1)..(2): phosphorothioate backbone
  misc_feature (2)..(3): phosphodiester backbone
  modified_base (2)..(2): 2'-O-(2-methoxyethyl)-modified thymidine
  misc_feature (3)..(4): phosphorothioate backbone
  modified_base (3)..(4): 2'-O-(2-methoxyethyl)-modified guanosine
  misc_feature (4)..(5): phosphodiester backbone
  misc_feature (5)..(6): phosphorothioate backbone
  misc_feature (6)..(7): phosphodiester backbone
  misc_feature (7)..(8): phosphorothioate backbone
  misc_feature (8)..(9): phosphodiester backbone
  misc_feature (9)..(10): phosphorothioate backbone
  misc_feature (10)..(11): phosphodiester backbone
  misc_feature (11)..(12): phosphorothioate backbone
  misc_feature (12)..(13): phosphodiester backbone
  misc_feature (13)..(14): phosphorothioate backbone
  misc_feature (14)..(15): phosphodiester backbone
  misc_feature (15)..(16): phosphorothioate backbone
  modified_base (15)..(16): 2'-O-(2-methoxyethyl)-modified 5-methylcytidine
  misc_feature (16)..(17): phosphodiester backbone
  misc_feature (17)..(18): phosphorothioate backbone
  modified_base (17)..(18): 2'-O-(2-methoxyethyl)-modified adenosine
nnnntgtcaacaagnnnn

SEQ ID NO: 390 - DNA, 17 bp, Artificial Sequence
  Synthetic Construct
  modified_base (1)..(1): locked nucleic acid thymidine
  misc_feature (1)..(17): phosphorothioate backbone
  modified_base (2)..(3): locked nucleic acid guanosine
  modified_base (14)..(15): locked nucleic acid 5-methylcytidine
  modified_base (16)..(17): locked nucleic acid adenosine
nnntgtcaacaagnnnn

SEQ ID NO: 391 - DNA, 17 bp, Artificial Sequence
  Synthetic Construct
  modified_base (1)..(1): locked nucleic acid thymidine
  misc_feature (1)..(3): phosphorothioate backbone
  modified_base (2)..(3): locked nucleic acid guanosine
  misc_feature (3)..(4): phosphodiester backbone
  misc_feature (4)..(13): phosphorothioate backbone
  misc_feature (13)..(14): phosphodiester backbone
  misc_feature (14)..(17): phosphorothioate backbone
  modified_base (14)..(15): locked nucleic acid 5-methylcytidine
  modified_base (16)..(17): locked nucleic acid adenosine
nnntgtcaacaagnnnn

SEQ ID NO: 392 - DNA, 17 bp, Artificial Sequence
  Synthetic Construct
  modified_base (1)..(1): locked nucleic acid thymidine
  misc_feature (1)..(2): phosphorothioate backbone
  misc_feature (2)..(3): phosphodiester backbone
  modified_base (2)..(3): locked nucleic acid guanosine
  misc_feature (3)..(4): phosphorothioate backbone
  misc_feature (4)..(5): phosphodiester backbone
  misc_feature (5)..(6): phosphorothioate backbone
  misc_feature (6)..(7): phosphodiester backbone
  misc_feature (7)..(8): phosphorothioate backbone
  misc_feature (8)..(9): phosphodiester backbone
  misc_feature (9)..(10): phosphorothioate backbone
  misc_feature (10)..(11): phosphodiester backbone
  misc_feature (11)..(12): phosphorothioate backbone
  misc_feature (12)..(13): phosphodiester backbone
  misc_feature (13)..(14): phosphorothioate backbone
  misc_feature (14)..(15): phosphodiester backbone
  modified_base (14)..(15): locked nucleic acid 5-methylcytidine
  misc_feature (15)..(16): phosphorothioate backbone
  misc_feature (16)..(17): phosphodiester backbone
  modified_base (16)..(17): locked nucleic acid adenosine
  misc_feature (17)..(18): phosphorothioate backbone
nnntgtcaacaagnnnn

SEQ ID NO: 393 - RNA, 20 nt, Artificial Sequence
  Synthetic Construct
gaaaccaucucugggauaag

SEQ ID NO: 394 - RNA, 20 nt, Artificial Sequence
  Synthetic Construct
aaaccaucucugggauaagg

SEQ ID NO: 395 - RNA, 20 nt, Artificial Sequence
  Synthetic Construct
aaccaucucugggauaagga

SEQ ID NO: 396 - RNA, 20 nt, Artificial Sequence
  Synthetic Construct
accaucucugggauaaggau

SEQ ID NO: 397 - RNA, 20 nt, Artificial Sequence
  Synthetic Construct
ccaucucugggauaaggaug

SEQ ID NO: 398 - RNA, 20 nt, Artificial Sequence
  Synthetic Construct
caucucugggauaaggauga

SEQ ID NO: 399 - RNA, 20 nt, Artificial Sequence
  Synthetic Construct
aucucugggauaaggaugac

SEQ ID NO: 400 - RNA, 20 nt, Artificial Sequence
  Synthetic Construct
ucucugggauaaggaugacu

SEQ ID NO: 401 - RNA, 20 nt, Artificial Sequence
  Synthetic Construct
cucugggauaaggaugacug

SEQ ID NO: 402 - RNA, 20 nt, Artificial Sequence
  Synthetic Construct
ucugggauaaggaugacuga

SEQ ID NO: 403 - RNA, 20 nt, Artificial Sequence
  Synthetic Construct
cugggauaaggaugacugag

SEQ ID NO: 404 - RNA, 20 nt, Artificial Sequence
  Synthetic Construct
ugggauaaggaugacugagg

SEQ ID NO: 405 - RNA, 20 nt, Artificial Sequence
  Synthetic Construct
gggauaaggaugacugagga

SEQ ID NO: 406 - RNA, 20 nt, Artificial Sequence
  Synthetic Construct
ggauaaggaugacugaggaa

SEQ ID NO: 407 - RNA, 20 nt, Artificial Sequence
  Synthetic Construct
gcugaaacaacugaaacuuc

SEQ ID NO: 408 - RNA, 20 nt, Artificial Sequence
  Synthetic Construct
gaaacaacugaaacuucagg

SEQ ID NO: 409 - RNA, 20 nt, Artificial Sequence
  Synthetic Construct
aaacaacugaaacuucaggg

SEQ ID NO: 410 - RNA, 20 nt, Artificial Sequence
  Synthetic Construct
aacaacugaaacuucaggga

SEQ ID NO: 411 - RNA, 20 nt, Artificial Sequence
  Synthetic Construct
acaacugaaacuucagggaa

SEQ ID NO: 412 - RNA, 20 nt, Artificial Sequence
  Synthetic Construct
caacugaaacuucagggaaa

SEQ ID NO: 413 - RNA, 20 nt, Artificial Sequence
  Synthetic Construct
acugaaacuucagggaaaag

SEQ ID NO: 414 - RNA, 19 nt, Artificial Sequence
  Synthetic Construct
aaccaucucugggauaagg

SEQ ID NO: 415 - RNA, 19 nt, Artificial Sequence
  Synthetic Construct
accaucucugggauaagga

SEQ ID NO: 416 - RNA, 19 nt, Artificial Sequence
  Synthetic Construct
ccaucucugggauaaggau

SEQ ID NO: 417 - RNA, 19 nt, Artificial Sequence
  Synthetic Construct
caucucugggauaaggaug

SEQ ID NO: 418 - RNA, 19 nt, Artificial Sequence
  Synthetic Construct
aucucugggauaaggauga

SEQ ID NO: 419 - RNA, 19 nt, Artificial Sequence
  Synthetic Construct
ucucugggauaaggaugac

SEQ ID NO: 420 - RNA, 19 nt, Artificial Sequence
  Synthetic Construct
cucugggauaaggaugacu

SEQ ID NO: 421 - RNA, 19 nt, Artificial Sequence
  Synthetic Construct
ucugggauaaggaugacug

SEQ ID NO: 422 - RNA, 19 nt, Artificial Sequence
  Synthetic Construct
cugggauaaggaugacuga

SEQ ID NO: 423 - RNA, 19 nt, Artificial Sequence
  Synthetic Construct
ugggauaaggaugacugag

SEQ ID NO: 424 - RNA, 19 nt, Artificial Sequence
  Synthetic Construct
gggauaaggaugacugagg

SEQ ID NO: 425 - RNA, 19 nt, Artificial Sequence
  Synthetic Construct
ggauaaggaugacugagga

SEQ ID NO: 426 - RNA, 19 nt, Artificial Sequence
  Synthetic Construct
aacaacugaaacuucaggg

SEQ ID NO: 427 - RNA, 19 nt, Artificial Sequence
  Synthetic Construct
acaacugaaacuucaggga

SEQ ID NO: 428 - RNA, 19 nt, Artificial Sequence
  Synthetic Construct
caacugaaacuucagggaa

SEQ ID NO: 429 - RNA, 19 nt, Artificial Sequence
  Synthetic Construct
caacugaaacuucagggaa

SEQ ID NO: 430 - RNA, 18 nt, Artificial Sequence
  Synthetic Construct
ccaucucugggauaagga

SEQ ID NO: 431 - RNA, 18 nt, Artificial Sequence
  Synthetic Construct
caucucugggauaaggau

SEQ ID NO: 432 - RNA, 18 nt, Artificial Sequence
  Synthetic Construct
aucucugggauaaggaug

SEQ ID NO: 433 - RNA, 18 nt, Artificial Sequence
  Synthetic Construct
ucucugggauaaggauga

SEQ ID NO: 434 - RNA, 18 nt, Artificial Sequence
  Synthetic Construct
cucugggauaaggaugac

SEQ ID NO: 435 - RNA, 18 nt, Artificial Sequence
  Synthetic Construct
ucugggauaaggaugacu

SEQ ID NO: 436 - RNA, 18 nt, Artificial Sequence
  Synthetic Construct
cugggauaaggaugacug

SEQ ID NO: 437 - RNA, 18 nt, Artificial Sequence
  Synthetic Construct
ugggauaaggaugacuga

SEQ ID NO: 438 - RNA, 18 nt, Artificial Sequence
  Synthetic Construct
gggauaaggaugacugag

SEQ ID NO: 439 - RNA, 18 nt, Artificial Sequence
  Synthetic Construct
ggauaaggaugacugagg

SEQ ID NO: 440 - RNA, 18 nt, Artificial Sequence
  Synthetic Construct
acaacugaaacuucaggg

SEQ ID NO: 441 - DNA, 20 bp, Artificial Sequence
  Synthetic Construct
cttatcccagagatggtttc

SEQ ID NO: 442 - DNA, 20 bp, Artificial Sequence
  Synthetic Construct
ccttatcccagagatggttt

SEQ ID NO: 443 - DNA, 20 bp, Artificial Sequence
  Synthetic Construct
tccttatcccagagatggtt

SEQ ID NO: 444 - DNA, 20 bp, Artificial Sequence
  Synthetic Construct
atccttatcccagagatggt

SEQ ID NO: 445 - DNA, 20 bp, Artificial Sequence
  Synthetic Construct
catccttatcccagagatgg

SEQ ID NO: 446 - DNA, 20 bp, Artificial Sequence
  Synthetic Construct
tcatccttatcccagagatg

SEQ ID NO: 447 - DNA, 20 bp, Artificial Sequence
  Synthetic Construct
gtcatccttatcccagagat

SEQ ID NO: 448 - DNA, 20 bp, Artificial Sequence
  Synthetic Construct
agtcatccttatcccagaga

SEQ ID NO: 449 - DNA, 20 bp, Artificial Sequence
  Synthetic Construct
cagtcatccttatcccagag

SEQ ID NO: 450 - DNA, 20 bp, Artificial Sequence
  Synthetic Construct
tcagtcatccttatcccaga

SEQ ID NO: 451 - DNA, 20 bp, Artificial Sequence
  Synthetic Construct
ctcagtcatccttatcccag

SEQ ID NO: 452 - DNA, 20 bp, Artificial Sequence
  Synthetic Construct
cctcagtcatccttatccca

SEQ ID NO: 453 - DNA, 20 bp, Artificial Sequence
  Synthetic Construct
tcctcagtcatccttatccc

SEQ ID NO: 454 - DNA, 20 bp, Artificial Sequence
  Synthetic Construct
ttcctcagtcatccttatcc

SEQ ID NO: 455 - DNA, 20 bp, Artificial Sequence
  Synthetic Construct
gaagtttcagttgtttcagc

SEQ ID NO: 456 - DNA, 20 bp, Artificial Sequence
  Synthetic Construct
cctgaagtttcagttgtttc

SEQ ID NO: 457 - DNA, 20 bp, Artificial Sequence
  Synthetic Construct
ccctgaagtttcagttgttt

SEQ ID NO: 458 - DNA, 20 bp, Artificial Sequence
  Synthetic Construct
tccctgaagtttcagttgtt

SEQ ID NO: 459 - DNA, 20 bp, Artificial Sequence
  Synthetic Construct
ttccctgaagtttcagttgt

SEQ ID NO: 460 - DNA, 20 bp, Artificial Sequence
  Synthetic Construct
tttccctgaagtttcagttg

SEQ ID NO: 461 - DNA, 20 bp, Artificial Sequence
  Synthetic Construct
cttttccctgaagtttcagt

SEQ ID NO: 462 - DNA, 19 bp, Artificial Sequence
  Synthetic Construct
ccttatcccagagatggtt

SEQ ID NO: 463 - DNA, 19 bp, Artificial Sequence
  Synthetic Construct
tccttatcccagagatggt

SEQ ID NO: 464 - DNA, 19 bp, Artificial Sequence
  Synthetic Construct
atccttatcccagagatgg

SEQ ID NO: 465 - DNA, 19 bp, Artificial Sequence
  Synthetic Construct
catccttatcccagagatg

SEQ ID NO: 466 - DNA, 19 bp, Artificial Sequence
  Synthetic Construct
tcatccttatcccagagat

SEQ ID NO: 467 - DNA, 19 bp, Artificial Sequence
  Synthetic Construct
gtcatccttatcccagaga

SEQ ID NO: 468 - DNA, 19 bp, Artificial Sequence
  Synthetic Construct
agtcatccttatcccagag

SEQ ID NO: 469 - DNA, 19 bp, Artificial Sequence
  Synthetic Construct
cagtcatccttatcccaga

SEQ ID NO: 470 - DNA, 19 bp, Artificial Sequence
  Synthetic Construct
tcagtcatccttatcccag

SEQ ID NO: 471 - DNA, 19 bp, Artificial Sequence
  Synthetic Construct
ctcagtcatccttatccca

SEQ ID NO: 472 - DNA, 19 bp, Artificial Sequence
  Synthetic Construct
cctcagtcatccttatccc

SEQ ID NO: 473 - DNA, 19 bp, Artificial Sequence
  Synthetic Construct
tcctcagtcatccttatcc

SEQ ID NO: 474 - DNA, 19 bp, Artificial Sequence
  Synthetic Construct
ccctgaagtttcagttgtt

SEQ ID NO: 475 - DNA, 19 bp, Artificial Sequence
  Synthetic Construct
tccctgaagtttcagttgt

SEQ ID NO: 476 - DNA, 19 bp, Artificial Sequence
  Synthetic Construct
ttccctgaagtttcagttg

SEQ ID NO: 477 - DNA, 19 bp, Artificial Sequence
  Synthetic Construct
ttccctgaagtttcagttg

SEQ ID NO: 478 - DNA, 18 bp, Artificial Sequence
  Synthetic Construct
tccttatcccagagatgg

SEQ ID NO: 479 - DNA, 18 bp, Artificial Sequence
  Synthetic Construct
atccttatcccagagatg

SEQ ID NO: 480 - DNA, 18 bp, Artificial Sequence
  Synthetic Construct
catccttatcccagagat

SEQ ID NO: 481 - DNA, 18 bp, Artificial Sequence
  Synthetic Construct
tcatccttatcccagaga

SEQ ID NO: 482 - DNA, 18 bp, Artificial Sequence
  Synthetic Construct
gtcatccttatcccagag

SEQ ID NO: 483 - DNA, 18 bp, Artificial Sequence
  Synthetic Construct
agtcatccttatcccaga

SEQ ID NO: 484 - DNA, 18 bp, Artificial Sequence
  Synthetic Construct
cagtcatccttatcccag

SEQ ID NO: 485 - DNA, 18 bp, Artificial Sequence
  Synthetic Construct
tcagtcatccttatccca

SEQ ID NO: 486 - DNA, 18 bp, Artificial Sequence
  Synthetic Construct
ctcagtcatccttatccc

SEQ ID NO: 487 - DNA, 18 bp, Artificial Sequence
  Synthetic Construct
cctcagtcatccttatcc

SEQ ID NO: 488 - DNA, 18 bp, Artificial Sequence
  Synthetic Construct
ccctgaagtttcagttgt

SEQ ID NO: 489 - DNA, 228 bp, Artificial Sequence
  Synthetic Construct
aatgaaatcttctgatttgtaagacatgctgccaagagattagttttacaccttcaggataaagactgctgagaaggtttaaggatgctattctgaaaagactgtggaggaagattaaggaaaccatctctgggataaggatgactgaggaaatttaaggatgccactctggttaaaagctgaaacaactgaaacttcagggaaaagagaaggcctggaatctgatcc

SEQ ID NO: 490 - DNA, 79 bp, Artificial Sequence
  Synthetic Construct
gggtcaatgatgacaacccaatgtcatgaagaaatgtgatgacataaaatttatgctcaataggattacgctgagtccc

SEQ ID NO: 491 - DNA, 79 bp, Artificial Sequence
  Synthetic Construct
gggtcaataatggcaatccaatgtcatgaagaaaggtgatgacataaaattcatgctcaataggattactctgaggccc

SEQ ID NO: 492 - DNA, 88 bp, Artificial Sequence
  Synthetic Construct
gggttcacaaagtgcaatccctcgagccaatgtcatgaagaaaggtgatgacataaaattcatgctcaataggattatgctgaggccc

SEQ ID NO: 493 - DNA, 79 bp, Artificial Sequence
  Synthetic Construct
ttgtcaatgataacaacccaaaatcatgaacagaggtgatgatataaaaatcatgctcaataggattacgctgaggcac

SEQ ID NO: 494 - DNA, 69 bp, Artificial Sequence
  Synthetic Construct
tggccatcataggtcatgaagagtggtgatgacattaaaatcatgatcaataggattacactgaggccc

SEQ ID NO: 495 - DNA, 82 bp, Artificial Sequence
  Synthetic Construct
gggtcaatgatgagaaccttatattgtcctgaagagcggtgatgacttaaaaatcatgctcaataggattacgctgaggccc

SEQ ID NO: 496 - DNA, 76 bp, Artificial Sequence
  Synthetic Construct
gggtcaatgatgagatgttaccttgaagagaaatgatgacgtaaaaattaagttcagttggattacgctgaggccc

SEQ ID NO: 497 - DNA, 53 bp, Artificial Sequence
  Synthetic Construct
ttatattgtcttcgacagggaagatgacataaaaattatgttcaataggatta

SEQ ID NO: 498 - DNA, 71 bp, Artificial Sequence
  Synthetic Construct
tcaataatgaaatcttctgatttggtgagaaataatgccttaaaattacactcaataggattatgctgagg

SEQ ID NO: 499 - DNA, 33 bp, Artificial Sequence
  Synthetic Construct
taaaaatcatgctcaatagaattaagctgaggc

SEQ ID NO: 500 - DNA, 20 bp, Artificial Sequence
  Synthetic Construct
atatgtggaagccggaatct

SEQ ID NO: 501 - DNA, 21 bp, Artificial Sequence
  Synthetic Construct
cccagaactccctaatcagaa

SEQ ID NO: 502 - DNA, 20 bp, Artificial Sequence
  Synthetic Construct
atgacggtggctataccagg

SEQ ID NO: 503 - DNA, 20 bp, Artificial Sequence
  Synthetic Construct
gtctccttcgagctgtttgc

SEQ ID NO: 504 - DNA, 21 bp, Artificial Sequence
  Synthetic Construct
cctttctctccagtgctcaga

SEQ ID NO: 505 - DNA, 21 bp, Artificial Sequence
  Synthetic Construct
cctgtgaactttcaaccagga

SEQ ID NO: 506 - DNA, 20 bp, Artificial Sequence
  Synthetic Construct
ggatcagactccaggccttc

SEQ ID NO: 507 - RNA, 20 nt, Artificial Sequence
  Synthetic Construct
cccagguguccuuuaaugaa

SEQ ID NO: 508 - RNA, 20 nt, Artificial Sequence
  Synthetic Construct
ccagguguccuuuaaugaaa

SEQ ID NO: 509 - RNA, 20 nt, Artificial Sequence
  Synthetic Construct
ugaaaaugcucuugacacca

SEQ ID NO: 510 - RNA, 20 nt, Artificial Sequence
  Synthetic Construct
gaaaaugcucuugacaccaa

SEQ ID NO: 511 - RNA, 20 nt, Artificial Sequence
  Synthetic Construct
aaaugcucuugacaccaaug

SEQ ID NO: 512 - RNA, 20 nt, Artificial Sequence
  Synthetic Construct
agaucaguagcuuccuuuac

SEQ ID NO: 513 - RNA, 20 nt, Artificial Sequence
  Synthetic Construct
ucaguagcuuccuuuaccga

SEQ ID NO: 514 - RNA, 20 nt, Artificial Sequence
  Synthetic Construct
ucuagaacauugagcuaugg

SEQ ID NO: 515 - RNA, 20 nt, Artificial Sequence
  Synthetic Construct
cuagaacauugagcuaugga

SEQ ID NO: 516 - skipped

SEQ ID NO: 517 - RNA, 20 nt, Artificial Sequence
  Synthetic Construct
acauugagcuauggaagacu

SEQ ID NO: 518 - RNA, 20 nt, Artificial Sequence
  Synthetic Construct
cuauggaagacucccaccua

SEQ ID NO: 519 - RNA, 20 nt, Artificial Sequence
  Synthetic Construct
uauggaagacucccaccuaa

SEQ ID NO: 520 - RNA, 20 nt, Artificial Sequence
  Synthetic Construct
caagugcuaccgcacaggca

SEQ ID NO: 521 - RNA, 20 nt, Artificial Sequence
  Synthetic Construct
aagugcuaccgcacaggcau

SEQ ID NO: 522 - RNA, 20 nt, Artificial Sequence
  Synthetic Construct
uaccgcacaggcaugcugca

SEQ ID NO: 523 - RNA, 20 nt, Artificial Sequence
  Synthetic Construct
caggcaugcugcagugaauu

SEQ ID NO: 524 - RNA, 20 nt, Artificial Sequence
  Synthetic Construct
aggcaugcugcagugaauuu

SEQ ID NO: 525 - RNA, 20 nt, Artificial Sequence
  Synthetic Construct
accguuguuuaaggaugcua

SEQ ID NO: 526 - RNA, 20 nt, Artificial Sequence
  Synthetic Construct
ccguuguuuaaggaugcuau

SEQ ID NO: 527 - RNA, 20 nt, Artificial Sequence
  Synthetic Construct
cuguggaggaagaaaacccu

SEQ ID NO: 528 - RNA, 20 nt, Artificial Sequence
  Synthetic Construct
aagaaaacccuuuacccugu

SEQ ID NO: 529 - RNA, 20 nt, Artificial Sequence
  Synthetic Construct
agaaaacccuuuacccuguu

SEQ ID NO: 530 - RNA, 20 nt, Artificial Sequence
  Synthetic Construct
cucaacugccuggcacugaa

SEQ ID NO: 531 - RNA, 20 nt, Artificial Sequence
  Synthetic Construct
aacugccuggcacugaaaau

SEQ ID NO: 532 - RNA, 20 nt, Artificial Sequence
  Synthetic Construct
acugccuggcacugaaaaug

SEQ ID NO: 533 - RNA, 20 nt, Artificial Sequence
  Synthetic Construct
guguuuaaggaaaccaucuc

SEQ ID NO: 534 - RNA, 20 nt, Artificial Sequence
  Synthetic Construct
guuuaaggaaaccaucucug

SEQ ID NO: 535 - RNA, 20 nt, Artificial Sequence
  Synthetic Construct
aggaaaccaucucugauaag

SEQ ID NO: 536 - RNA, 20 nt, Artificial Sequence
  Synthetic Construct
ucuuuggcuuguugacacca

SEQ ID NO: 537 - RNA, 20 nt, Artificial Sequence
  Synthetic Construct
cuuuggcuuguugacaccag

SEQ ID NO: 538 - DNA, 20 bp, Artificial Sequence
  Synthetic Construct
ttcattaaaggacacctggg

SEQ ID NO: 539 - DNA, 20 bp, Artificial Sequence
  Synthetic Construct
tttcattaaaggacacctgg

SEQ ID NO: 540 - DNA, 20 bp, Artificial Sequence
  Synthetic Construct
tggtgtcaagagcattttca

SEQ ID NO: 541 - DNA, 20 bp, Artificial Sequence
  Synthetic Construct
ttggtgtcaagagcattttc

SEQ ID NO: 542 - DNA, 20 bp, Artificial Sequence
  Synthetic Construct
cattggtgtcaagagcattt

SEQ ID NO: 543 - DNA, 20 bp, Artificial Sequence
  Synthetic Construct
gtaaaggaagctactgatct

SEQ ID NO: 544 - DNA, 20 bp, Artificial Sequence
  Synthetic Construct
tcggtaaaggaagctactga

SEQ ID NO: 545 - DNA, 20 bp, Artificial Sequence
  Synthetic Construct
ccatagctcaatgttctaga

SEQ ID NO: 546 - DNA, 20 bp, Artificial Sequence
  Synthetic Construct
tccatagctcaatgttctag

SEQ ID NO: 547 - DNA, 20 bp, Artificial Sequence
  Synthetic Construct
gtcttccatagctcaatgtt

SEQ ID NO: 548 - DNA, 20 bp, Artificial Sequence
  Synthetic Construct
agtcttccatagctcaatgt

SEQ ID NO: 549 - DNA, 20 bp, Artificial Sequence
  Synthetic Construct
taggtgggagtcttccatag

SEQ ID NO: 550 - DNA, 20 bp, Artificial Sequence
  Synthetic Construct
ttaggtgggagtcttccata

SEQ ID NO: 551 - DNA, 20 bp, Artificial Sequence
  Synthetic Construct
tgcctgtgcggtagcacttg

SEQ ID NO: 552 - DNA, 20 bp, Artificial Sequence
  Synthetic Construct
atgcctgtgcggtagcactt

SEQ ID NO: 553 - DNA, 20 bp, Artificial Sequence
  Synthetic Construct
tgcagcatgcctgtgcggta

SEQ ID NO: 554 - DNA, 20 bp, Artificial Sequence
  Synthetic Construct
aattcactgcagcatgcctg

SEQ ID NO: 555 - DNA, 20 bp, Artificial Sequence
  Synthetic Construct
aaattcactgcagcatgcct

SEQ ID NO: 556 - DNA, 20 bp, Artificial Sequence
  Synthetic Construct
tagcatccttaaacaacggt

SEQ ID NO: 557 - DNA, 20 bp, Artificial Sequence
  Synthetic Construct
atagcatccttaaacaacgg

SEQ ID NO: 558 - DNA, 20 bp, Artificial Sequence
  Synthetic Construct
agggttttcttcctccacag

SEQ ID NO: 559 - DNA, 20 bp, Artificial Sequence
  Synthetic Construct
acagggtaaagggttttctt

SEQ ID NO: 560 - DNA, 20 bp, Artificial Sequence
  Synthetic Construct
aacagggtaaagggttttct

SEQ ID NO: 561 - DNA, 20 bp, Artificial Sequence
  Synthetic Construct
ttcagtgccaggcagttgag

SEQ ID NO: 562 - DNA, 20 bp, Artificial Sequence
  Synthetic Construct
attttcagtgccaggcagtt

SEQ ID NO: 563 - DNA, 20 bp, Artificial Sequence
  Synthetic Construct
cattttcagtgccaggcagt

SEQ ID NO: 564 - DNA, 20 bp, Artificial Sequence
  Synthetic Construct
gagatggtttccttaaacac

SEQ ID NO: 565 - DNA, 20 bp, Artificial Sequence
  Synthetic Construct
cagagatggtttccttaaac

SEQ ID NO: 566 - DNA, 20 bp, Artificial Sequence
  Synthetic Construct
cttatcagagatggtttcct

SEQ ID NO: 567 - DNA, 20 bp, Artificial Sequence
  Synthetic Construct
tggtgtcaacaagccaaaga

SEQ ID NO: 568 - DNA, 20 bp, Artificial Sequence
  Synthetic Construct
ctggtgtcaacaagccaaag

SEQ ID NO: 569 - DNA, 58 bp, Artificial Sequence
  Synthetic Construct
ggtgccattctattataaataacctgacccattatttataatagaatggcaccttttt

SEQ ID NO: 570 - DNA, 58 bp, Artificial Sequence
  Synthetic Construct
gctttcatcaataatgaaataacctgacccattatttcattattgatgaaagcttttt

SEQ ID NO: 571 - DNA, 58 bp, Artificial Sequence
  Synthetic Construct
ggtctttcatcaataatgataacctgacccattatcattattgatgaaagaccttttt

SEQ ID NO: 572 - DNA, 58 bp, Artificial Sequence
  Synthetic Construct
gaaatcttctgatttgtaataacctgacccattattacaaatcagaagatttcttttt

SEQ ID NO: 573 - DNA, 58 bp, Artificial Sequence
  Synthetic Construct
gcacctaagggaattagtataacctgacccattatactaattcccttaggtgcttttt

SEQ ID NO: 574 - DNA, 58 bp, Artificial Sequence
  Synthetic Construct
gtttcaaccaggatttaaataacctgacccattatttaaatcctggttgaaacttttt

SEQ ID NO: 575 - DNA, 58 bp, Artificial Sequence
  Synthetic Construct
gctttcaaccaggatttaataacctgacccattattaaatcctggttgaaagcttttt

SEQ ID NO: 576 - DNA, 58 bp, Artificial Sequence
  Synthetic Construct
ggagatgtgccattctatataacctgacccattatatagaatggcacatctccttttt

SEQ ID NO: 577 - DNA, 58 bp, Artificial Sequence
  Synthetic Construct
gtctttcatcaataatgaataacctgacccattattcattattgatgaaagacttttt

SEQ ID NO: 578 - DNA, 58 bp, Artificial Sequence
  Synthetic Construct
gatcaataatgaaatcttataacctgacccattataagatttcattattgatcttttt

SEQ ID NO: 579 - DNA, 58 bp, Artificial Sequence
  Synthetic Construct
gtgtctttcatcaataatataacctgacccattatattattgatgaaagacacttttt

SEQ ID NO: 580 - DNA, 58 bp, Artificial Sequence
  Synthetic Construct
gcaataatgaaatcttctataacctgacccattatagaagatttcattattgcttttt

SEQ ID NO: 581 - DNA, 58 bp, Artificial Sequence
  Synthetic Construct
gcatgctgcagtgaatttataacctgacccattataaattcactgcagcatgcttttt

SEQ ID NO: 582 - DNA, 58 bp, Artificial Sequence
  Synthetic Construct
ggaaatcttctgatttgtataacctgacccattatacaaatcagaagatttccttttt

SEQ ID NO: 583 - DNA, 58 bp, Artificial Sequence
  Synthetic Construct
ggtatattctatctagaaataacctgacccattatttctagatagaatataccttttt

SEQ ID NO: 584 - DNA, 58 bp, Artificial Sequence
  Synthetic Construct
gtgctgcagtgaatttaaataacctgacccattatttaaattcactgcagcacttttt

SEQ ID NO: 585 - DNA, 58 bp, Artificial Sequence
  Synthetic Construct
gtgtgccattctattataataacctgacccattattataatagaatggcacacttttt

SEQ ID NO: 586 - DNA, 58 bp, Artificial Sequence
  Synthetic Construct
gttaccatcagtgtttaaataacctgacccattatttaaacactgatggtaacttttt

SEQ ID NO: 587 - DNA, 58 bp, Artificial Sequence
  Synthetic Construct
gcctgcaaccgttgtttaataacctgacccattattaaacaacggttgcaggcttttt

SEQ ID NO: 588 - DNA, 58 bp, Artificial Sequence
  Synthetic Construct
gtatgtctttcatcaataataacctgacccattattattgatgaaagacatacttttt

SEQ ID NO: 589 - DNA, 20 bp, Artificial Sequence
  Synthetic Construct
acactgatggtaaagtggac

SEQ ID NO: 590 - DNA, 20 bp, Artificial Sequence
  Synthetic Construct
tagaatatacacgtcggtaa

SEQ ID NO: 591 - DNA, 20 bp, Artificial Sequence
  Synthetic Construct
tcaactgtcccagtcacaac

SEQ ID NO: 592 - DNA, 20 bp, Artificial Sequence
  Synthetic Construct
tctagatagaatatacacgt

SEQ ID NO: 593 - DNA, 20 bp, Artificial Sequence
  Synthetic Construct
tctagatagaatatacacgt

SEQ ID NO: 594 - DNA, 20 bp, Artificial Sequence
  Synthetic Construct
ctccccatgcacacttgaga

SEQ ID NO: 595 - DNA, 20 bp, Artificial Sequence
  Synthetic Construct
catccttaaacaacggttgc

SEQ ID NO: 596 - DNA, 20 bp, Artificial Sequence
  Synthetic Construct
ggtgtaaaactaattccctt

SEQ ID NO: 597 - DNA, 20 bp, Artificial Sequence
  Synthetic Construct
aacaacggttgcagggacag

SEQ ID NO: 598 - DNA, 20 bp, Artificial Sequence
  Synthetic Construct
tatggaagactcccacctaa

SEQ ID NO: 599 - DNA, 20 bp, Artificial Sequence
  Synthetic Construct
ctatggaagactcccaccta

SEQ ID NO: 600 - DNA, 20 bp, Artificial Sequence
  Synthetic Construct
aagccttctcaagtgtgcat

SEQ ID NO: 601 - DNA, 20 bp, Artificial Sequence
  Synthetic Construct
ctatctagaacattgagcta

SEQ ID NO: 602 - DNA, 20 bp, Artificial Sequence
  Synthetic Construct
accctctggtgttgtcacag

SEQ ID NO: 603 - DNA, 20 bp, Artificial Sequence
  Synthetic Construct
aaccctttaccctgttgttc